European Patent Specification EP 3 978 522 B1, published October 1, 2025. Title: HUMAN ANTIBODIES TO FEL D1 AND METHODS OF USE THEREOF. Applicant: Regeneron Pharmaceuticals, Inc. Application To be assigned. The sequence listing filed with the application follows.

SEQUENCE LISTING (490 sequences)

SEQ ID NO: 1 - DNA, 363 bp, Artificial Sequence
  Synthetic
gaggtgcagctggtggagtctgggggaggcttggtccagcctggggggtccctgagactctcctgtacagcctctggattcatttttagtaacttttggatgacttgggtccgccaggctccagggaaggggctggagtgggtggccaacataaagcaagatggaagtgagacatactgtgtggactctgtgaagggccgattcaccatctccagagaccacgccaagaactcactgtttctgcaaatgaacagcctgagagccgaggacacggctgtatattactgtgcaagaggagctggaacaatctactactacggtatggacgtctggggccaagggaccacggtcattgtctcctca

SEQ ID NO: 2 - protein, 121 aa, Artificial Sequence
  Synthetic
EVQLVESGGGLVQPGGSLRLSCTASGFIFSNFWMTWVRQAPGKGLEWVANIKQDGSETYCVDSVKGRFTISRDHAKNSLFLQMNSLRAEDTAVYYCARGAGTIYYYGMDVWGQGTTVIVSS

SEQ ID NO: 3 - DNA, 24 bp, Artificial Sequence
  Synthetic
ggattcatttttagtaacttttgg

SEQ ID NO: 4 - protein, 8 aa, Artificial Sequence
  Synthetic
GFIFSNFW

SEQ ID NO: 5 - DNA, 24 bp, Artificial Sequence
  Synthetic
ataaagcaagatggaagtgagaca

SEQ ID NO: 6 - protein, 8 aa, Artificial Sequence
  Synthetic
IKQDGSET

SEQ ID NO: 7 - DNA, 42 bp, Artificial Sequence
  Synthetic
gcaagaggagctggaacaatctactactacggtatggacgtc

SEQ ID NO: 8 - protein, 14 aa, Artificial Sequence
  Synthetic
ARGAGTIYYYGMDV

SEQ ID NO: 9 - DNA, 321 bp, Artificial Sequence
  Synthetic
gacatccagatgacccagtctccatcttccgtgtctgcatctgtaggagacagactcaccatcacttgtcgggcgagtcaggatattagcagctggttaacctggtatcagcagaaaccagggaaagcccctaacctcctgatctatgctgcatccggtttgcaaagtggagtcccatcaaggttcagcggcagtggatctgggacagatttcactctcaccatcagcaacctgcagcctgaagattttgcaacttactattgtcaacaggctaacagtttcccgctcaccttcggccaagggacacgactggagattaaa

SEQ ID NO: 10 - protein, 107 aa, Artificial Sequence
  Synthetic
DIQMTQSPSSVSASVGDRLTITCRASQDISSWLTWYQQKPGKAPNLLIYAASGLQSGVPSRFSGSGSGTDFTLTISNLQPEDFATYYCQQANSFPLTFGQGTRLEIK

SEQ ID NO: 11 - DNA, 18 bp, Artificial Sequence
  Synthetic
caggatattagcagctgg

SEQ ID NO: 12 - protein, 6 aa, Artificial Sequence
  Synthetic
QDISSW

SEQ ID NO: 13 - DNA, 9 bp, Artificial Sequence
  Synthetic
gctgcatcc

SEQ ID NO: 14 - protein, 3 aa, Artificial Sequence
  Synthetic
AAS

SEQ ID NO: 15 - DNA, 27 bp, Artificial Sequence
  Synthetic
caacaggctaacagtttcccgctcacc

SEQ ID NO: 16 - protein, 9 aa, Artificial Sequence
  Synthetic
QQANSFPLT

SEQ ID NO: 17 - DNA, 357 bp, Artificial Sequence
  Synthetic
gaggtgcagctggtggagtctgggggaggcctggtcaagcctggggggtccctgagactctcctgtgcagcctctggattcaccttcagaaactataacataaactgggtccgccaggctccagggaaggggctggagtgggtctcactcatcagtggtagtagtagttacatatattacgcagactcagtgaagggccgattcaccgtctccagagacaacgccaagaactcactgtatctgcaaatgaacagcctgagagccgaggacacggctgtgtattactgtgcgaggcggacattaagctactacgttatggacgtctggggccaagggaccacggtcaccgtctcctca

SEQ ID NO: 18 - protein, 119 aa, Artificial Sequence
  Synthetic
EVQLVESGGGLVKPGGSLRLSCAASGFTFRNYNINWVRQAPGKGLEWVSLISGSSSYIYYADSVKGRFTVSRDNAKNSLYLQMNSLRAEDTAVYYCARRTLSYYVMDVWGQGTTVTVSS

SEQ ID NO: 19 - DNA, 24 bp, Artificial Sequence
  Synthetic
ggattcaccttcagaaactataac

SEQ ID NO: 20 - protein, 8 aa, Artificial Sequence
  Synthetic
GFTFRNYN

SEQ ID NO: 21 - DNA, 24 bp, Artificial Sequence
  Synthetic
atcagtggtagtagtagttacata

SEQ ID NO: 22 - protein, 8 aa, Artificial Sequence
  Synthetic
ISGSSSYI

SEQ ID NO: 23 - DNA, 36 bp, Artificial Sequence
  Synthetic
gcgaggcggacattaagctactacgttatggacgtc

SEQ ID NO: 24 - protein, 12 aa, Artificial Sequence
  Synthetic
ARRTLSYYVMDV

SEQ ID NO: 25 - DNA, 321 bp, Artificial Sequence
  Synthetic
gacatccaggtgacccagtctccatcccccctgtctgcatctgtaggagacagagtcaccatcacttgccgggcgagtcagggcattagcaattatttagcctggtatcagcagaaaccagggagagttcctcagctcctgatctatgctgcatccactttgcaatcaggggtcccatctcggttcagtggcagtggatctgggacagatttcactctcaccatcagcagcctgcagcctgaagatgttgcaacttattactgtcaaaagtataacagtgccccgtacacttttggccaggggaccaagctggagatcaaa

SEQ ID NO: 26 - protein, 107 aa, Artificial Sequence
  Synthetic
DIQVTQSPSPLSASVGDRVTITCRASQGISNYLAWYQQKPGRVPQLLIYAASTLQSGVPSRFSGSGSGTDFTLTISSLQPEDVATYYCQKYNSAPYTFGQGTKLEIK

SEQ ID NO: 27 - DNA, 18 bp, Artificial Sequence
  Synthetic
cagggcattagcaattat

SEQ ID NO: 28 - protein, 6 aa, Artificial Sequence
  Synthetic
QGISNY

SEQ ID NO: 29 - DNA, 9 bp, Artificial Sequence
  Synthetic
gctgcatcc

SEQ ID NO: 30 - protein, 3 aa, Artificial Sequence
  Synthetic
AAS

SEQ ID NO: 31 - DNA, 27 bp, Artificial Sequence
  Synthetic
caaaagtataacagtgccccgtacact

SEQ ID NO: 32 - protein, 9 aa, Artificial Sequence
  Synthetic
QKYNSAPYT

SEQ ID NO: 33 - DNA, 363 bp, Artificial Sequence
  Synthetic
caggtacagctgcagcagtcaggtccaggactggtgaagtcctcgcagaccctctcactcacctgtgccatctccggggacagtgtctctagcaacagtgttgcttggaattggatcaggcagtccccatcgagaggccttgagtggctggggaggacatactacaggtccaaatggtataatgattatgcagtatctgtgaaaagtcgaataaacatcaacccagacacatccaagaaccacttctccctgcagttgaattctgtgactcccgaggacacggctgtttatttctgtgcaagagcctggaactggtactaccttgactactggggccagggcaccctggtcaccgtctcgtca

SEQ ID NO: 34 - protein, 121 aa, Artificial Sequence
  Synthetic
QVQLQQSGPGLVKSSQTLSLTCAISGDSVSSNSVAWNWIRQSPSRGLEWLGRTYYRSKWYNDYAVSVKSRININPDTSKNHFSLQLNSVTPEDTAVYFCARAWNWYYLDYWGQGTLVTVSS

SEQ ID NO: 35 - DNA, 30 bp, Artificial Sequence
  Synthetic
ggggacagtgtctctagcaacagtgttgct

SEQ ID NO: 36 - protein, 10 aa, Artificial Sequence
  Synthetic
GDSVSSNSVA

SEQ ID NO: 37 - DNA, 27 bp, Artificial Sequence
  Synthetic
acatactacaggtccaaatggtataat

SEQ ID NO: 38 - protein, 9 aa, Artificial Sequence
  Synthetic
TYYRSKWYN

SEQ ID NO: 39 - DNA, 33 bp, Artificial Sequence
  Synthetic
gcaagagcctggaactggtactaccttgactac

SEQ ID NO: 40 - protein, 11 aa, Artificial Sequence
  Synthetic
ARAWNWYYLDY

SEQ ID NO: 41 - DNA, 339 bp, Artificial Sequence
  Synthetic
gatattgtgatgacccagtctccagactccctggctatgtctctaggcgagagggccaccatcaactgcaagtccagccagagtgttttatacagctccaacaataagaattacttaggttggtaccagcagaaaccaggacagcctcctaaactgctcatttactgggcatctacccgggaatccggtgtccctgaccgaatcagtggcagcgggtctgggacagatttcactctcaccatcagcagcctgcaggctgaagatgtggcagtttattactgtcagcaatatcttagaaatacgctcactttcggcggagggaccaaggtggagatcaaa

SEQ ID NO: 42 - protein, 113 aa, Artificial Sequence
  Synthetic
DIVMTQSPDSLAMSLGERATINCKSSQSVLYSSNNKNYLGWYQQKPGQPPKLLIYWASTRESGVPDRISGSGSGTDFTLTISSLQAEDVAVYYCQQYLRNTLTFGGGTKVEIK

SEQ ID NO: 43 - DNA, 36 bp, Artificial Sequence
  Synthetic
cagagtgttttatacagctccaacaataagaattac

SEQ ID NO: 44 - protein, 12 aa, Artificial Sequence
  Synthetic
QSVLYSSNNKNY

SEQ ID NO: 45 - DNA, 9 bp, Artificial Sequence
  Synthetic
tgggcatct

SEQ ID NO: 46 - protein, 3 aa, Artificial Sequence
  Synthetic
WAS

SEQ ID NO: 47 - DNA, 27 bp, Artificial Sequence
  Synthetic
cagcaatatcttagaaatacgctcact

SEQ ID NO: 48 - protein, 9 aa, Artificial Sequence
  Synthetic
QQYLRNTLT

SEQ ID NO: 49 - DNA, 381 bp, Artificial Sequence
  Synthetic
gaggtgcagctggtggagtctgggggaggcctggtcaagcctggggggtccctgagactctcctgtgcagcctctggattcaccttcagtagctatagcatgaactgggtccgccaggctccagggaaggggctggagtgggtctcatccattagtagtagaagtagttacatatactacgcagactcagtgaagggccgattcaccatctcaagagacaacgccaagaactcactgtatctgcaaatgaacagcctgagagccgaggacacggctgtgtattattgtgcgagagatcatattgtagtagtaccaggtgcctcctactactactacggtatggacgtctggggccaagggaccacggtcaccgtctcctca

SEQ ID NO: 50 - protein, 127 aa, Artificial Sequence
  Synthetic
EVQLVESGGGLVKPGGSLRLSCAASGFTFSSYSMNWVRQAPGKGLEWVSSISSRSSYIYYADSVKGRFTISRDNAKNSLYLQMNSLRAEDTAVYYCARDHIVVVPGASYYYYGMDVWGQGTTVTVSS

SEQ ID NO: 51 - DNA, 24 bp, Artificial Sequence
  Synthetic
ggattcaccttcagtagctatagc

SEQ ID NO: 52 - protein, 8 aa, Artificial Sequence
  Synthetic
GFTFSSYS

SEQ ID NO: 53 - DNA, 24 bp, Artificial Sequence
  Synthetic
attagtagtagaagtagttacata

SEQ ID NO: 54 - protein, 8 aa, Artificial Sequence
  Synthetic
ISSRSSYI

SEQ ID NO: 55 - DNA, 60 bp, Artificial Sequence
  Synthetic
gcgagagatcatattgtagtagtaccaggtgcctcctactactactacggtatggacgtc

SEQ ID NO: 56 - protein, 20 aa, Artificial Sequence
  Synthetic
ARDHIVVVPGASYYYYGMDV

SEQ ID NO: 57 - DNA, 321 bp, Artificial Sequence
  Synthetic
gacatccagatgacccagtctccatcctccctgtctgcatctgtaggagacagagtcaccatcacttgccgggcaagtcagggcattagaaatgatttaggctggtatcagcagaaaccagggaaagcccctaagcgcctgatctctgctgcatccagtttgcaaagtggggtcccatcaaggttcagcggcagtggatctgggacagaattcactctcacaatcagcagcctgcagcctgaagattttgcaacttattactgtctacagcataatagttacccgctcactttcggcggagggaccaaggtggagatcaaa

SEQ ID NO: 58 - protein, 107 aa, Artificial Sequence
  Synthetic
DIQMTQSPSSLSASVGDRVTITCRASQGIRNDLGWYQQKPGKAPKRLISAASSLQSGVPSRFSGSGSGTEFTLTISSLQPEDFATYYCLQHNSYPLTFGGGTKVEIK

SEQ ID NO: 59 - DNA, 18 bp, Artificial Sequence
  Synthetic
cagggcattagaaatgat

SEQ ID NO: 60 - protein, 6 aa, Artificial Sequence
  Synthetic
QGIRND

SEQ ID NO: 61 - DNA, 9 bp, Artificial Sequence
  Synthetic
gctgcatcc

SEQ ID NO: 62 - protein, 3 aa, Artificial Sequence
  Synthetic
AAS

SEQ ID NO: 63 - DNA, 27 bp, Artificial Sequence
  Synthetic
ctacagcataatagttacccgctcact

SEQ ID NO: 64 - protein, 9 aa, Artificial Sequence
  Synthetic
LQHNSYPLT

SEQ ID NO: 65 - DNA, 369 bp, Artificial Sequence
  Synthetic
caggtgcagctggtgcagtctggggctgaggtgaagaagcctggggcctcagtggaggtctcctgcaaggcttctggatacaccttcaccgactactatatacactggatacgacaggcccctggacaagggcttgagtggatgggatggatcaaccctgacagtggtcgcacaaactatgcacagaagtttcaggtcagggtcaccatgaccagggacacgtccatcaccacagcctacatggaactgaacagactgaaatctgacgacacggccgtgtattactgtgcgagaggacccctacgtggatatagcggctacgatttttttgactactggggccagggaaccctggtcaccgtctcctca

SEQ ID NO: 66 - protein, 123 aa, Artificial Sequence
  Synthetic
QVQLVQSGAEVKKPGASVEVSCKASGYTFTDYYIHWIRQAPGQGLEWMGWINPDSGRTNYAQKFQVRVTMTRDTSITTAYMELNRLKSDDTAVYYCARGPLRGYSGYDFFDYWGQGTLVTVSS

SEQ ID NO: 67 - DNA, 24 bp, Artificial Sequence
  Synthetic
ggatacaccttcaccgactactat

SEQ ID NO: 68 - protein, 8 aa, Artificial Sequence
  Synthetic
GYTFTDYY

SEQ ID NO: 69 - DNA, 24 bp, Artificial Sequence
  Synthetic
atcaaccctgacagtggtcgcaca

SEQ ID NO: 70 - protein, 8 aa, Artificial Sequence
  Synthetic
INPDSGRT

SEQ ID NO: 71 - DNA, 48 bp, Artificial Sequence
  Synthetic
gcgagaggacccctacgtggatatagcggctacgatttttttgactac

SEQ ID NO: 72 - protein, 16 aa, Artificial Sequence
  Synthetic
ARGPLRGYSGYDFFDY

SEQ ID NO: 73 - DNA, 339 bp, Artificial Sequence
  Synthetic
gacatcgtgatgacccagtctccagactccctggctatatctctgggcgagagggccaccatcaactgcaagtccagccagagtgttttatacagctccaacaataagcagtacttagcttggtacaagcagagaccaggacagcctcctaagctgctcatttcctggacatctacccgggaatccggggtccctgaccgattcagtggcagcgggtctgggacagatttcactctcaccatcagcagcctgcaggctgaagatgtggcagtttatttctgtcaacaatattatagtactccgtacacttttggccaggggaccaagctggagatcaga

SEQ ID NO: 74 - protein, 113 aa, Artificial Sequence
  Synthetic
DIVMTQSPDSLAISLGERATINCKSSQSVLYSSNNKQYLAWYKQRPGQPPKLLISWTSTRESGVPDRFSGSGSGTDFTLTISSLQAEDVAVYFCQQYYSTPYTFGQGTKLEIR

SEQ ID NO: 75 - DNA, 36 bp, Artificial Sequence
  Synthetic
cagagtgttttatacagctccaacaataagcagtac

SEQ ID NO: 76 - protein, 12 aa, Artificial Sequence
  Synthetic
QSVLYSSNNKQY

SEQ ID NO: 77 - DNA, 9 bp, Artificial Sequence
  Synthetic
tggacatct

SEQ ID NO: 78 - protein, 3 aa, Artificial Sequence
  Synthetic
WTS

SEQ ID NO: 79 - DNA, 27 bp, Artificial Sequence
  Synthetic
caacaatattatagtactccgtacact

SEQ ID NO: 80 - protein, 9 aa, Artificial Sequence
  Synthetic
QQYYSTPYT

SEQ ID NO: 81 - DNA, 369 bp, Artificial Sequence
  Synthetic
caggtggtactggtggagtctgggggaggcgtggtccagcctgggaggtccctgagactctcctgtgcagcgtctggattcaccttcagtagctatggcatgcactgggtccgccaggctccaggcaaggggctggagtgggtggcagttatatggtatgatggaagtaataaatactatgtagactccgtgaagggccgattcaccatctccagagacaattccaataacacaatctatctgcaaatgaacagcctgagagccgaggacacggctgtatattactgtgcgagatcccttataccagtggctggtacggaccccatttttggatactggggccagggaaccctggtcaccgtctcctca

SEQ ID NO: 82 - protein, 123 aa, Artificial Sequence
  Synthetic
QVVLVESGGGVVQPGRSLRLSCAASGFTFSSYGMHWVRQAPGKGLEWVAVIWYDGSNKYYVDSVKGRFTISRDNSNNTIYLQMNSLRAEDTAVYYCARSLIPVAGTDPIFGYWGQGTLVTVSS

SEQ ID NO: 83 - DNA, 24 bp, Artificial Sequence
  Synthetic
ggattcaccttcagtagctatggc

SEQ ID NO: 84 - protein, 8 aa, Artificial Sequence
  Synthetic
GFTFSSYG

SEQ ID NO: 85 - DNA, 24 bp, Artificial Sequence
  Synthetic
atatggtatgatggaagtaataaa

SEQ ID NO: 86 - protein, 8 aa, Artificial Sequence
  Synthetic
IWYDGSNK

SEQ ID NO: 87 - DNA, 48 bp, Artificial Sequence
  Synthetic
gcgagatcccttataccagtggctggtacggaccccatttttggatac

SEQ ID NO: 88 - protein, 16 aa, Artificial Sequence
  Synthetic
ARSLIPVAGTDPIFGY

SEQ ID NO: 89 - DNA, 321 bp, Artificial Sequence
  Synthetic
gacatccagatgacccagtctccttccaccctgtctgcatctgtaggagacagagtcaccatcacttgccgggccagtcagagtgttagtagctggttggcctggtatcagcagaaaccagggaaagcccctaaactcctgatctttaaggcgtctggtttagaaagtggggtcccatttaggttcagcggcagtggatctgggacagaattcactctcaccatcagcagcctgcagcctgatgattttgcaacttattactgccaacagtataatacttattctccgacgttcggccaagggaccaaggtggagatcaaa

SEQ ID NO: 90 - protein, 107 aa, Artificial Sequence
  Synthetic
DIQMTQSPSTLSASVGDRVTITCRASQSVSSWLAWYQQKPGKAPKLLIFKASGLESGVPFRFSGSGSGTEFTLTISSLQPDDFATYYCQQYNTYSPTFGQGTKVEIK

SEQ ID NO: 91 - DNA, 18 bp, Artificial Sequence
  Synthetic
cagagtgttagtagctgg

SEQ ID NO: 92 - protein, 6 aa, Artificial Sequence
  Synthetic
QSVSSW

SEQ ID NO: 93 - DNA, 9 bp, Artificial Sequence
  Synthetic
aaggcgtct

SEQ ID NO: 94 - protein, 3 aa, Artificial Sequence
  Synthetic
KAS

SEQ ID NO: 95 - DNA, 27 bp, Artificial Sequence
  Synthetic
caacagtataatacttattctccgacg

SEQ ID NO: 96 - protein, 9 aa, Artificial Sequence
  Synthetic
QQYNTYSPT

SEQ ID NO: 97 - DNA, 360 bp, Artificial Sequence
  Synthetic
caggtgcagctgcaggagtcgggcccaggactggtgaagccttcggagaccctgtccctcacctgcactgtctctggtggctccatcagtaattactactggagctggatccggcagcccccagggaagggactggagtggattggatatatctattatagtgggagaaccaactacaacccctccctcaagagtcgagtcaccatatcagtggacacgtccaagaaccagttctccctgaagctgaggtctgtgaccgccgcagacacggccgtgtattactgtgcgagacatcgtataactagaactgcggactcctttgactactggggccagggaaccctggtcaccgtctcctca

SEQ ID NO: 98 - protein, 120 aa, Artificial Sequence
  Synthetic
QVQLQESGPGLVKPSETLSLTCTVSGGSISNYYWSWIRQPPGKGLEWIGYIYYSGRTNYNPSLKSRVTISVDTSKNQFSLKLRSVTAADTAVYYCARHRITRTADSFDYWGQGTLVTVSS

SEQ ID NO: 99 - DNA, 24 bp, Artificial Sequence
  Synthetic
ggtggctccatcagtaattactac

SEQ ID NO: 100 - protein, 8 aa, Artificial Sequence
  Synthetic
GGSISNYY

SEQ ID NO: 101 - DNA, 21 bp, Artificial Sequence
  Synthetic
atctattatagtgggagaacc

SEQ ID NO: 102 - protein, 7 aa, Artificial Sequence
  Synthetic
IYYSGRT

SEQ ID NO: 103 - DNA, 42 bp, Artificial Sequence
  Synthetic
gcgagacatcgtataactagaactgcggactcctttgactac

SEQ ID NO: 104 - protein, 14 aa, Artificial Sequence
  Synthetic
ARHRITRTADSFDY

SEQ ID NO: 105 - DNA, 321 bp, Artificial Sequence
  Synthetic
gacatccagatgacccagtctccatcctccctgtctgcatctgtaggagacagagtcaccatcacttgccaggcgagtcaggacattaccaactatttaaattggtatcagcagaaaccagggaaagcccctaagctcctgatctacgatgcatccaatttggaaacaggggtcccatcaaggttcagtggaagtggatctgggacagattttactttcaccatcagcagcctgcagcctgaagatgttgcaacattttactgtcaccagtatggtgatctcccgtacacttttggccaggggaccaagctggagatcaaa

SEQ ID NO: 106 - protein, 107 aa, Artificial Sequence
  Synthetic
DIQMTQSPSSLSASVGDRVTITCQASQDITNYLNWYQQKPGKAPKLLIYDASNLETGVPSRFSGSGSGTDFTFTISSLQPEDVATFYCHQYGDLPYTFGQGTKLEIK

SEQ ID NO: 107 - DNA, 18 bp, Artificial Sequence
  Synthetic
caggacattaccaactat

SEQ ID NO: 108 - protein, 6 aa, Artificial Sequence
  Synthetic
QDITNY

SEQ ID NO: 109 - DNA, 9 bp, Artificial Sequence
  Synthetic
gatgcatcc

SEQ ID NO: 110 - protein, 3 aa, Artificial Sequence
  Synthetic
DAS

SEQ ID NO: 111 - DNA, 27 bp, Artificial Sequence
  Synthetic
caccagtatggtgatctcccgtacact

SEQ ID NO: 112 - protein, 9 aa, Artificial Sequence
  Synthetic
HQYGDLPYT

SEQ ID NO: 113 - DNA, 369 bp, Artificial Sequence
  Synthetic
caggtggtattggtggagtctgggggaggcgtggtccagcctgggaggtccctgagactctcctgtgcagcgtctggattcaccttcagtagctatggcatgcactgggtccgccaggctccaggcaaggggctggagtgggtggcagttatttggtatgatggaagtattaaatactatgcagactccgtgaagggccgattcaccatctccagagacaattccaataacacaatctatctgcaaatgaacagcctgagagccgaggacacggctgtatattactgtgcgagagcccttataccagtggctggtacggaccccatttttgggtactggggccagggaaccctggtcaccgtctcctca

SEQ ID NO: 114 - protein, 123 aa, Artificial Sequence
  Synthetic
QVVLVESGGGVVQPGRSLRLSCAASGFTFSSYGMHWVRQAPGKGLEWVAVIWYDGSIKYYADSVKGRFTISRDNSNNTIYLQMNSLRAEDTAVYYCARALIPVAGTDPIFGYWGQGTLVTVSS

SEQ ID NO: 115 - DNA, 24 bp, Artificial Sequence
  Synthetic
ggattcaccttcagtagctatggc

SEQ ID NO: 116 - protein, 8 aa, Artificial Sequence
  Synthetic
GFTFSSYG

SEQ ID NO: 117 - DNA, 24 bp, Artificial Sequence
  Synthetic
atttggtatgatggaagtattaaa

SEQ ID NO: 118 - protein, 8 aa, Artificial Sequence
  Synthetic
IWYDGSIK

SEQ ID NO: 119 - DNA, 48 bp, Artificial Sequence
  Synthetic
gcgagagcccttataccagtggctggtacggaccccatttttgggtac

SEQ ID NO: 120 - protein, 16 aa, Artificial Sequence
  Synthetic
ARALIPVAGTDPIFGY

SEQ ID NO: 121 - DNA, 321 bp, Artificial Sequence
  Synthetic
gacatccagatgacccagtctccttccaccctgtctgcatctgtaggagacagagtcaccatcacttgccgggccagtcagagtgttagtagctggttggcctggtatcagcagaaaccagggaaagcccctaaactcctgatctttaagacgtctggtttagaaagtggggtcccatttaggttcagcggcagtggatctgggacagaattcactctcaccatcagcagcctgcagcctgatgattttgcaacttattactgccaacagtataatacttattctccgacgttcggccaagggaccaaggtggagatcaaa

SEQ ID NO: 122 - protein, 107 aa, Artificial Sequence
  Synthetic
DIQMTQSPSTLSASVGDRVTITCRASQSVSSWLAWYQQKPGKAPKLLIFKTSGLESGVPFRFSGSGSGTEFTLTISSLQPDDFATYYCQQYNTYSPTFGQGTKVEIK

SEQ ID NO: 123 - DNA, 18 bp, Artificial Sequence
  Synthetic
cagagtgttagtagctgg

SEQ ID NO: 124 - protein, 6 aa, Artificial Sequence
  Synthetic
QSVSSW

SEQ ID NO: 125 - DNA, 9 bp, Artificial Sequence
  Synthetic
aagacgtct

SEQ ID NO: 126 - protein, 3 aa, Artificial Sequence
  Synthetic
KTS

SEQ ID NO: 127 - DNA, 27 bp, Artificial Sequence
  Synthetic
caacagtataatacttattctccgacg

SEQ ID NO: 128 - protein, 9 aa, Artificial Sequence
  Synthetic
QQYNTYSPT

SEQ ID NO: 129 - DNA, 360 bp, Artificial Sequence
  Synthetic
caggtgcagctgcaggagtcgggcccaggactggtgaagccttcggagaccctgtccctcacctgcactgtctctggtggctccatcagtagttactactggagctggatccggcagcccccagggaagggactggagtggattggatatatctattacagtgggagaaccaactacaacccctccctcaagagtcgagtcaccatatcagtggacacgtccaagaaccagttctccctgaaactgagctctgtgaccgccgcagacacggccatttattactgtgcgagacatcgtgtaactagaactgcggactcctttgactactggggccagggaaccctggtcaccgtctcctca

SEQ ID NO: 130 - protein, 120 aa, Artificial Sequence
  Synthetic
QVQLQESGPGLVKPSETLSLTCTVSGGSISSYYWSWIRQPPGKGLEWIGYIYYSGRTNYNPSLKSRVTISVDTSKNQFSLKLSSVTAADTAIYYCARHRVTRTADSFDYWGQGTLVTVSS

SEQ ID NO: 131 - DNA, 24 bp, Artificial Sequence
  Synthetic
ggtggctccatcagtagttactac

SEQ ID NO: 132 - protein, 8 aa, Artificial Sequence
  Synthetic
GGSISSYY

SEQ ID NO: 133 - DNA, 21 bp, Artificial Sequence
  Synthetic
atctattacagtgggagaacc

SEQ ID NO: 134 - protein, 7 aa, Artificial Sequence
  Synthetic
IYYSGRT

SEQ ID NO: 135 - DNA, 42 bp, Artificial Sequence
  Synthetic
gcgagacatcgtgtaactagaactgcggactcctttgactac

SEQ ID NO: 136 - protein, 14 aa, Artificial Sequence
  Synthetic
ARHRVTRTADSFDY

SEQ ID NO: 137 - DNA, 321 bp, Artificial Sequence
  Synthetic
gacatccagatgacccagtctccatcctccctgtctgcatctgtaggagacagagtcaccatcacttgccaggcgagtcaggacattaacaactatttaaattggtatcagcagaaaacagggaaagcccctaagttcctgatctacgatgcatccaatttggaaacaggggtctcatcaaggttcagtggaagtggatctgggacagattttactttcaccatcagcagcctgcagcctgaagatgttggaacatattactgtcaccagtatggtgatctcccgtacacttttggccaggggaccaagctggagatcaaa

SEQ ID NO: 138 - protein, 107 aa, Artificial Sequence
  Synthetic
DIQMTQSPSSLSASVGDRVTITCQASQDINNYLNWYQQKTGKAPKFLIYDASNLETGVSSRFSGSGSGTDFTFTISSLQPEDVGTYYCHQYGDLPYTFGQGTKLEIK

SEQ ID NO: 139 - DNA, 18 bp, Artificial Sequence
  Synthetic
caggacattaacaactat

SEQ ID NO: 140 - protein, 6 aa, Artificial Sequence
  Synthetic
QDINNY

SEQ ID NO: 141 - DNA, 9 bp, Artificial Sequence
  Synthetic
gatgcatcc

SEQ ID NO: 142 - protein, 3 aa, Artificial Sequence
  Synthetic
DAS

SEQ ID NO: 143 - DNA, 27 bp, Artificial Sequence
  Synthetic
caccagtatggtgatctcccgtacact

SEQ ID NO: 144 - protein, 9 aa, Artificial Sequence
  Synthetic
HQYGDLPYT

SEQ ID NO: 145 - DNA, 360 bp, Artificial Sequence
  Synthetic
gaggtgcagctggtggagtctgggggaggcctggtcaggccggggggatccctgagactctcctgtgcagcctctggattcaccttcactagctatgccatgaattgggtccgccaggctccagggaagggactggagtgggtctcatccatttctagttatagttcttacatatatatcgcagactcagtgaagggccgattcaccctctccagagacaatgccaagaactcactgtatctacaaatgcacagtctgagacccgaggacacggctgtttatttctgtgcgagagagggatatagtgcctactcctactttgacttctggggccggggaaccctggtcaccgtctcctca

SEQ ID NO: 146 - protein, 120 aa, Artificial Sequence
  Synthetic
EVQLVESGGGLVRPGGSLRLSCAASGFTFTSYAMNWVRQAPGKGLEWVSSISSYSSYIYIADSVKGRFTLSRDNAKNSLYLQMHSLRPEDTAVYFCAREGYSAYSYFDFWGRGTLVTVSS

SEQ ID NO: 147 - DNA, 24 bp, Artificial Sequence
  Synthetic
ggattcaccttcactagctatgcc

SEQ ID NO: 148 - protein, 8 aa, Artificial Sequence
  Synthetic
GFTFTSYA

SEQ ID NO: 149 - DNA, 24 bp, Artificial Sequence
  Synthetic
atttctagttatagttcttacata

SEQ ID NO: 150 - protein, 8 aa, Artificial Sequence
  Synthetic
ISSYSSYI

SEQ ID NO: 151 - DNA, 39 bp, Artificial Sequence
  Synthetic
gcgagagagggatatagtgcctactcctactttgacttc

SEQ ID NO: 152 - protein, 13 aa, Artificial Sequence
  Synthetic
AREGYSAYSYFDF

SEQ ID NO: 153 - DNA, 321 bp, Artificial Sequence
  Synthetic
gacatccagatgacccagtctccttccaccctgtctgcatctgttggagacagagtcaccatcacttgccgggccagtcagagtgttattagttggttggcctggtatcaacagaaaccagggaaagcccctaaactcctgatccatagggcgtctagtttagaaagtggggtcccatcaaggttcagcggcagtggatctgggacagaattcactctcaccatcagcggcctgcagcctgatgattttgcaacttattactgtcaacagtataatacttattttccgacgttcggccaagggaccaaggtggaagtcaaa

SEQ ID NO: 154 - protein, 107 aa, Artificial Sequence
  Synthetic
DIQMTQSPSTLSASVGDRVTITCRASQSVISWLAWYQQKPGKAPKLLIHRASSLESGVPSRFSGSGSGTEFTLTISGLQPDDFATYYCQQYNTYFPTFGQGTKVEVK

SEQ ID NO: 155 - DNA, 18 bp, Artificial Sequence
  Synthetic
cagagtgttattagttgg

SEQ ID NO: 156 - protein, 6 aa, Artificial Sequence
  Synthetic
QSVISW

SEQ ID NO: 157 - DNA, 9 bp, Artificial Sequence
  Synthetic
agggcgtct

SEQ ID NO: 158 - protein, 3 aa, Artificial Sequence
  Synthetic
RAS

SEQ ID NO: 159 - DNA, 27 bp, Artificial Sequence
  Synthetic
caacagtataatacttattttccgacg

SEQ ID NO: 160 - protein, 9 aa, Artificial Sequence
  Synthetic
QQYNTYFPT

SEQ ID NO: 161 - DNA, 354 bp, Artificial Sequence
  Synthetic
gaggtggaactgttggaatctgggggaggcttggtacagcctggggggtccctgagactctcctgtgcagcctctggattcacctttagtagttatgccatgagttgggtccgccaggctccagggaaggggctggagtgggtctcatctattagtggtagggttggtagcacacatttcgcagactccgtgaagggccggttcaccttctccagagacaattccaagaacacgctgtatctgcagctgagcagcctgagagccgaggacacggccgtatattactgtgcgagaagtagaggagcagcctactttgactactggggccagggaaccctggtcaccgtctcctca

SEQ ID NO: 162 - protein, 118 aa, Artificial Sequence
  Synthetic
EVELLESGGGLVQPGGSLRLSCAASGFTFSSYAMSWVRQAPGKGLEWVSSISGRVGSTHFADSVKGRFTFSRDNSKNTLYLQLSSLRAEDTAVYYCARSRGAAYFDYWGQGTLVTVSS

SEQ ID NO: 163 - DNA, 24 bp, Artificial Sequence
  Synthetic
ggattcacctttagtagttatgcc

SEQ ID NO: 164 - protein, 8 aa, Artificial Sequence
  Synthetic
GFTFSSYA

SEQ ID NO: 165 - DNA, 24 bp, Artificial Sequence
  Synthetic
attagtggtagggttggtagcaca

SEQ ID NO: 166 - protein, 8 aa, Artificial Sequence
  Synthetic
ISGRVGST

SEQ ID NO: 167 - DNA, 33 bp, Artificial Sequence
  Synthetic
gcgagaagtagaggagcagcctactttgactac

SEQ ID NO: 168 - protein, 11 aa, Artificial Sequence
  Synthetic
ARSRGAAYFDY

SEQ ID NO: 169 - DNA, 321 bp, Artificial Sequence
  Synthetic
gacatccagatgacccagtctccatcctccctgtctgcatctgtaggagacagagtcaccatcacttgccaggcgaatcaggacattagcaactttttaaattggtatcagcagagaccagggaaagcccctaacctcctgatctatgctgcatccaatttggaaacaggggtcccatcaaggttcagtggaagtggatctgggacagattttactttcaccatcagcagcctgcagcctgaagatattgcaacatattactgtcaacattatgataattttccattcactttcggccctgggaccaaggtggatatcaaa

SEQ ID NO: 170 - protein, 107 aa, Artificial Sequence
  Synthetic
DIQMTQSPSSLSASVGDRVTITCQANQDISNFLNWYQQRPGKAPNLLIYAASNLETGVPSRFSGSGSGTDFTFTISSLQPEDIATYYCQHYDNFPFTFGPGTKVDIK

SEQ ID NO: 171 - DNA, 18 bp, Artificial Sequence
  Synthetic
caggacattagcaacttt

SEQ ID NO: 172 - protein, 6 aa, Artificial Sequence
  Synthetic
QDISNF

SEQ ID NO: 173 - DNA, 9 bp, Artificial Sequence
  Synthetic
gctgcatcc

SEQ ID NO: 174 - protein, 3 aa, Artificial Sequence
  Synthetic
AAS

SEQ ID NO: 175 - DNA, 27 bp, Artificial Sequence
  Synthetic
caacattatgataattttccattcact

SEQ ID NO: 176 - protein, 9 aa, Artificial Sequence
  Synthetic
QHYDNFPFT

SEQ ID NO: 177 - DNA, 363 bp, Artificial Sequence
  Synthetic
cagctgcagctgcaggagtcgggcccaggactggtgaacccttcggagaccctgtccctcacctgctctgtctctggtggctccatcagcagtgttaattactactggggctggatccgccagtccccagggaagggactggagtggattgggagtatctattatactgggagtaccgactacaacccgtccctcaagaatcgagtcaccatatccgtagacacgtccaagaaccagttctccctgaagcagacttctgtgaccgccgcagacacggctgtctattactgtgcgagacatgtggcactggctgggggggcttttgatatctggggccaggggacaatggtcaccgtctcttca

SEQ ID NO: 178 - protein, 121 aa, Artificial Sequence
  Synthetic
QLQLQESGPGLVNPSETLSLTCSVSGGSISSVNYYWGWIRQSPGKGLEWIGSIYYTGSTDYNPSLKNRVTISVDTSKNQFSLKQTSVTAADTAVYYCARHVALAGGAFDIWGQGTMVTVSS

SEQ ID NO: 179 - DNA, 30 bp, Artificial Sequence
  Synthetic
ggtggctccatcagcagtgttaattactac

SEQ ID NO: 180 - protein, 10 aa, Artificial Sequence
  Synthetic
GGSISSVNYY

SEQ ID NO: 181 - DNA, 21 bp, Artificial Sequence
  Synthetic
atctattatactgggagtacc

SEQ ID NO: 182 - protein, 7 aa, Artificial Sequence
  Synthetic
IYYTGST

SEQ ID NO: 183 - DNA, 39 bp, Artificial Sequence
  Synthetic
gcgagacatgtggcactggctgggggggcttttgatatc

SEQ ID NO: 184 - protein, 13 aa, Artificial Sequence
  Synthetic
ARHVALAGGAFDI

SEQ ID NO: 185 - DNA, 315 bp, Artificial Sequence
  Synthetic
gaaattgtgttgacgcagtctccaggcaccctgtctttgtctccaggggaaagagccaccctctcctgcagggccagtcagagtgttagtagcagcttcttaggctggtaccaacagaaacctggccaggctcccaggctcctcatctatggttcttccaccagggccactggcatcccagacaggttcagtggcagtgggtctgggacagacttcaatatcaccatcagcagactggagcctgaagattttgcagtgtattactgtcagcagtttggtaggtccttcggccctgggaccaagctggagatcaaa

SEQ ID NO: 186 - protein, 105 aa, Artificial Sequence
  Synthetic
EIVLTQSPGTLSLSPGERATLSCRASQSVSSSFLGWYQQKPGQAPRLLIYGSSTRATGIPDRFSGSGSGTDFNITISRLEPEDFAVYYCQQFGRSFGPGTKLEIK

SEQ ID NO: 187 - DNA, 21 bp, Artificial Sequence
  Synthetic
cagagtgttagtagcagcttc

SEQ ID NO: 188 - protein, 7 aa, Artificial Sequence
  Synthetic
QSVSSSF

SEQ ID NO: 189 - DNA, 9 bp, Artificial Sequence
  Synthetic
ggttcttcc

SEQ ID NO: 190 - protein, 3 aa, Artificial Sequence
  Synthetic
GSS

SEQ ID NO: 191 - DNA, 18 bp, Artificial Sequence
  Synthetic
cagcagtttggtaggtcc

SEQ ID NO: 192 - protein, 6 aa, Artificial Sequence
  Synthetic
QQFGRS

SEQ ID NO: 193 - DNA, 360 bp, Artificial Sequence
  Synthetic
caggtgcagctggtggagtctgggggaggcttggtcaagcctggagggtccctgagactctcctgcgcagcctctggattcaccttcagtgactattacatgaactggatccgccaggctccagggaaggggctggagtggatttcatatattagtagtggtggtagtaccacatactacgcagactctgtgaagggccgattcaccatctccagggacaacgccaagaactcactgtatctgcaaatgaacagcctgagagccgaggacacggccgtgtattactgtgcgagagatgggaagtacaacacctcgccgggggactactggggccagggaaccctggtcaccgtctcctca

SEQ ID NO: 194 - protein, 120 aa, Artificial Sequence
  Synthetic
QVQLVESGGGLVKPGGSLRLSCAASGFTFSDYYMNWIRQAPGKGLEWISYISSGGSTTYYADSVKGRFTISRDNAKNSLYLQMNSLRAEDTAVYYCARDGKYNTSPGDYWGQGTLVTVSS

SEQ ID NO: 195 - DNA, 24 bp, Artificial Sequence
  Synthetic
ggattcaccttcagtgactattac

SEQ ID NO: 196 - protein, 8 aa, Artificial Sequence
  Synthetic
GFTFSDYY

SEQ ID NO: 197 - DNA, 24 bp, Artificial Sequence
  Synthetic
attagtagtggtggtagtaccaca

SEQ ID NO: 198 - protein, 8 aa, Artificial Sequence
  Synthetic
ISSGGSTT

SEQ ID NO: 199 - DNA, 39 bp, Artificial Sequence
  Synthetic
gcgagagatgggaagtacaacacctcgccgggggactac

SEQ ID NO: 200 - protein, 13 aa, Artificial Sequence
  Synthetic
ARDGKYNTSPGDY

SEQ ID NO: 201 - DNA, 318 bp, Artificial Sequence
  Synthetic
gaaattgtgttgacgcagtctccagactttcagtctgtgactccaaaggagaaagtcaccatcacctgccgggccagtcagtccattggtagtagcttacactggtaccagcagaaaccagatcagtctccaaagctcctcatcaagtatgcttcccagtccttctcaggggtcccctcgaggttcagtggcagtggatctgggacagatttcaccctcaccatcaatagcctggaagctgaagatgctgctacgtattactgtcttcagagtagtagtttacggacgttcggccaagggaccaaagtggatatcaaa

SEQ ID NO: 202 - protein, 106 aa, Artificial Sequence
  Synthetic
EIVLTQSPDFQSVTPKEKVTITCRASQSIGSSLHWYQQKPDQSPKLLIKYASQSFSGVPSRFSGSGSGTDFTLTINSLEAEDAATYYCLQSSSLRTFGQGTKVDIK

SEQ ID NO: 203 - DNA, 18 bp, Artificial Sequence
  Synthetic
cagtccattggtagtagc

SEQ ID NO: 204 - protein, 6 aa, Artificial Sequence
  Synthetic
QSIGSS

SEQ ID NO: 205 - DNA, 9 bp, Artificial Sequence
  Synthetic
tatgcttcc

SEQ ID NO: 206 - protein, 3 aa, Artificial Sequence
  Synthetic
YAS

SEQ ID NO: 207 - DNA, 24 bp, Artificial Sequence
  Synthetic
cttcagagtagtagtttacggacg

SEQ ID NO: 208 - protein, 8 aa, Artificial Sequence
  Synthetic
LQSSSLRT

SEQ ID NO: 209 - DNA, 360 bp, Artificial Sequence
  Synthetic
caggtgcagctggtggagtctgggggaggcttggtcaagcctggagggtccctgagactctcctgtgcagcctctggattcaccttcagtgactactacatgaactggatccgccaggctccagggaaggggctggagtggatttcatacattagtagtagtggtagtaccacatactacgcagactctgtgaagggccgattcaccatctccagggacaacgccaagaactcactgtttctgcaaatgaacagcctgagaggcgaggacacggccgtgtattattgtgcgagagatgggagatacaacaccgtcgccggggactactggggccagggaaccacggtcaccgtctcctca

SEQ ID NO: 210 - protein, 120 aa, Artificial Sequence
  Synthetic
QVQLVESGGGLVKPGGSLRLSCAASGFTFSDYYMNWIRQAPGKGLEWISYISSSGSTTYYADSVKGRFTISRDNAKNSLFLQMNSLRGEDTAVYYCARDGRYNTVAGDYWGQGTTVTVSS

SEQ ID NO: 211 - DNA, 24 bp, Artificial Sequence
  Synthetic
ggattcaccttcagtgactactac

SEQ ID NO: 212 - protein, 8 aa, Artificial Sequence
  Synthetic
GFTFSDYY

SEQ ID NO: 213 - DNA, 24 bp, Artificial Sequence
  Synthetic
attagtagtagtggtagtaccaca

SEQ ID NO: 214 - protein, 8 aa, Artificial Sequence
  Synthetic
ISSSGSTT

SEQ ID NO: 215 - DNA, 39 bp, Artificial Sequence
  Synthetic
gcgagagatgggagatacaacaccgtcgccggggactac

SEQ ID NO: 216 - protein, 13 aa, Artificial Sequence
  Synthetic
ARDGRYNTVAGDY

SEQ ID NO: 217 - DNA, 321 bp, Artificial Sequence
  Synthetic
gaaattgtgatgacgcagtctccagactttcagtctgtggctccaaaggagaaagtcaccatcacctgccgggccagtcagaacattggtggtagcttacactggtaccagcagaaaccagatcagtctccaaagctcctcatcaagtatgcttcccagtccttctcaggggtcccctcgaggttcagtggcagtggatctgggacagatttcaccctcaccatcaatagcctggaagctgaagatgctgcaacgtattactgtcttcagagttacactttacggacgttcggccaagggaccaaggtggagatcaaacga

SEQ ID NO: 218 - protein, 107 aa, Artificial Sequence
  Synthetic
EIVMTQSPDFQSVAPKEKVTITCRASQNIGGSLHWYQQKPDQSPKLLIKYASQSFSGVPSRFSGSGSGTDFTLTINSLEAEDAATYYCLQSYTLRTFGQGTKVEIKR

SEQ ID NO: 219 - DNA, 18 bp, Artificial Sequence
  Synthetic
cagaacattggtggtagc

SEQ ID NO: 220 - protein, 6 aa, Artificial Sequence
  Synthetic
QNIGGS

SEQ ID NO: 221 - DNA, 9 bp, Artificial Sequence
  Synthetic
tatgcttcc

SEQ ID NO: 222 - protein, 3 aa, Artificial Sequence
  Synthetic
YAS

SEQ ID NO: 223 - DNA, 24 bp, Artificial Sequence
  Synthetic
cttcagagttacactttacggacg

SEQ ID NO: 224 - protein, 8 aa, Artificial Sequence
  Synthetic
LQSYTLRT

SEQ ID NO: 225 - DNA, 360 bp, Artificial Sequence
  Synthetic
gaggtgcagctggtggagtctgggggaggcttggtcaagcctggagggtccctgagactctcctgtgcagcctctggattcaccttcagtgactactacatgaactggatccgccaggctccagggaaggggctggagtgggtttcatatattagtagtagtggcagcagtatttattacgcagactctgtgaagggccgattcaccatctccagggacaacgccaagaactcactgtatctgctaatgaacagcctgagagccgaggacacggccgtgtattactgtgcgagagatgggaagtataacagttcgccgggggactactggggccagggaaccctggtcaccgtctcctca

SEQ ID NO: 226 - protein, 120 aa, Artificial Sequence
  Synthetic
EVQLVESGGGLVKPGGSLRLSCAASGFTFSDYYMNWIRQAPGKGLEWVSYISSSGSSIYYADSVKGRFTISRDNAKNSLYLLMNSLRAEDTAVYYCARDGKYNSSPGDYWGQGTLVTVSS

SEQ ID NO: 227 - DNA, 24 bp, Artificial Sequence
  Synthetic
ggattcaccttcagtgactactac

SEQ ID NO: 228 - protein, 8 aa, Artificial Sequence
  Synthetic
GFTFSDYY

SEQ ID NO: 229 - DNA, 24 bp, Artificial Sequence
  Synthetic
attagtagtagtggcagcagtatt

SEQ ID NO: 230 - protein, 8 aa, Artificial Sequence
  Synthetic
ISSSGSSI

SEQ ID NO: 231 - DNA, 39 bp, Artificial Sequence
  Synthetic
gcgagagatgggaagtataacagttcgccgggggactac

SEQ ID NO: 232 - protein, 13 aa, Artificial Sequence
  Synthetic
ARDGKYNSSPGDY

SEQ ID NO: 233 - DNA, 324 bp, Artificial Sequence
  Synthetic
gacatccagatgacccagtctccatcctcactgtctgcatctgtaggagacagagtcaccatcgcttgtcgggcgagtcagggcattagcaattatttagcctggtttcagcagaaaccagggaaagcccctaagtccctgatctatgctgcatccagtttgcaaagtggggtcccatcaaagttcagcggcagtggatctgggacagatttcactctcaccatcagcagcctgcagcctgaagattttgcaacttattactgccaacagtataacagttacccgctcactttcggcggagggaccaaggtggaaatcaaacga

SEQ ID NO: 234 - protein, 108 aa, Artificial Sequence
  Synthetic
DIQMTQSPSSLSASVGDRVTIACRASQGISNYLAWFQQKPGKAPKSLIYAASSLQSGVPSKFSGSGSGTDFTLTISSLQPEDFATYYCQQYNSYPLTFGGGTKVEIKR

SEQ ID NO: 235 - DNA, 18 bp, Artificial Sequence
  Synthetic
cagggcattagcaattat

SEQ ID NO: 236 - protein, 6 aa, Artificial Sequence
  Synthetic
QGISNY

SEQ ID NO: 237 - DNA, 9 bp, Artificial Sequence
  Synthetic
gctgcatcc

SEQ ID NO: 238 - protein, 3 aa, Artificial Sequence
  Synthetic
AAS

SEQ ID NO: 239 - DNA, 27 bp, Artificial Sequence
  Synthetic
caacagtataacagttacccgctcact

SEQ ID NO: 240 - protein, 9 aa, Artificial Sequence
  Synthetic
QQYNSYPLT

SEQ ID NO: 241 - DNA, 360 bp, Artificial Sequence
  Synthetic
gaggtgcagctggtggagtctgggggaggcttggtcaagcctggagggtccctgagactctcctgtgcagcctctggattcaccttcagtgactactacatgaactggatccgccaggctccagggaaggggctggagtgggtttcatatattagtagtagtggcagtagtatttattacgcagactctgtgaagggccgattcaccatctccagggacaacgccaagaactcactgtatctgctaatgaacagcctgagagccgaggacacggccgtgtattactgtgcgagagatgggaagtataacagctcgccgggggactactggggccagggaaccctggtcactgtctcctca

SEQ ID NO: 242 - protein, 120 aa, Artificial Sequence; identical to SEQ ID NO: 226
  Synthetic

SEQ ID NO: 243 - DNA, 24 bp, Artificial Sequence
  Synthetic
ggattcaccttcagtgactactac

SEQ ID NO: 244 - protein, 8 aa, Artificial Sequence
  Synthetic
GFTFSDYY

SEQ ID NO: 245 - DNA, 24 bp, Artificial Sequence
  Synthetic
attagtagtagtggcagtagtatt

SEQ ID NO: 246 - protein, 8 aa, Artificial Sequence
  Synthetic
ISSSGSSI

SEQ ID NO: 247 - DNA, 39 bp, Artificial Sequence
  Synthetic
gcgagagatgggaagtataacagctcgccgggggactac

SEQ ID NO: 248 - protein, 13 aa, Artificial Sequence
  Synthetic
ARDGKYNSSPGDY

SEQ ID NO: 249 - DNA, 318 bp, Artificial Sequence
  Synthetic
gaaattgtgctgactcagtctccagactttcagtctgtgactccaaaggagaaagtcaccatcacctgccgggccagtcagagcattggtggtagcttacactggtaccagcagaaaccagatcagtctccaaagctcctcatcaagtatgcttcccagtccttctcaggggtcccctcgaggttcagtggcagtggatctgggacagatttcaccctcaccatcaatagcctggaagctgaagatgctgcaacgtattactgtcttcagagtagtagtttacggacgttcggccaagggaccaaggtggaaatcaaa

SEQ ID NO: 250 - protein, 106 aa, Artificial Sequence
  Synthetic
EIVLTQSPDFQSVTPKEKVTITCRASQSIGGSLHWYQQKPDQSPKLLIKYASQSFSGVPSRFSGSGSGTDFTLTINSLEAEDAATYYCLQSSSLRTFGQGTKVEIK

SEQ ID NO: 251 - DNA, 18 bp, Artificial Sequence
  Synthetic
cagagcattggtggtagc

SEQ ID NO: 252 - protein, 6 aa, Artificial Sequence
  Synthetic
QSIGGS

SEQ ID NO: 253 - DNA, 9 bp, Artificial Sequence
  Synthetic
tatgcttcc

SEQ ID NO: 254 - protein, 3 aa, Artificial Sequence
  Synthetic
YAS

SEQ ID NO: 255 - DNA, 24 bp, Artificial Sequence
  Synthetic
cttcagagtagtagtttacggacg

SEQ ID NO: 256 - protein, 8 aa, Artificial Sequence
  Synthetic
LQSSSLRT

SEQ ID NO: 257 - DNA, 363 bp, Artificial Sequence
  Synthetic
gaggtgcagctggtggagtctgggggaggcttggtcaagcctggagggtccctgagactctcctgtgcagcctctggattcaccttcagtgactactacatgaactggatccgccaggctccagggaaggggctggagtgggtttcatacattagtagtagtggtaattccatatactacgcagactctgtgaagggccgattcaccatctccagggacaacgccaagaactcactgtttctgcagatgagcagcctgagagccgaggacacggccgtgtattactgtgcgagagatgggaggtataacgaccgtcgccgggggtactactggggccagggaaccctggtcaccgtctcctca

SEQ ID NO: 258 - protein, 121 aa, Artificial Sequence
  Synthetic
EVQLVESGGGLVKPGGSLRLSCAASGFTFSDYYMNWIRQAPGKGLEWVSYISSSGNSIYYADSVKGRFTISRDNAKNSLFLQMSSLRAEDTAVYYCARDGRYNDRRRGYYWGQGTLVTVSS

SEQ ID NO: 259 - DNA, 24 bp, Artificial Sequence
  Synthetic
ggattcaccttcagtgactactac

SEQ ID NO: 260 - protein, 8 aa, Artificial Sequence
  Synthetic
GFTFSDYY

SEQ ID NO: 261 - DNA, 24 bp, Artificial Sequence
  Synthetic
attagtagtagtggtaattccata

SEQ ID NO: 262 - protein, 8 aa, Artificial Sequence
  Synthetic
ISSSGNSI

SEQ ID NO: 263 - DNA, 42 bp, Artificial Sequence
  Synthetic
gcgagagatgggaggtataacgaccgtcgccgggggtactac

SEQ ID NO: 264 - protein, 14 aa, Artificial Sequence
  Synthetic
ARDGRYNDRRRGYY

SEQ ID NO: 265 - DNA, 321 bp, Artificial Sequence
  Synthetic
gaaattgtgatgacgcagtctccagactttcagtctgtgactccaaaggagaaagtcaccatcacctgccgggccagtcagagcattggtagtagcttacactggtaccagcagaaaccagatcagtctccaaaactcctcatcaagtatgcttcccagtccttctcaggggtcccctcgaggttcagtggcagtggatctgggacagatttcaccctcaccatcaatagcctggaagctgaagatgctgcaacgtattactgtcttcagagtagtagtttacggacgttcggccaagggaccaaggtggagatcaaacga

SEQ ID NO: 266 - protein, 107 aa, Artificial Sequence
  Synthetic
EIVMTQSPDFQSVTPKEKVTITCRASQSIGSSLHWYQQKPDQSPKLLIKYASQSFSGVPSRFSGSGSGTDFTLTINSLEAEDAATYYCLQSSSLRTFGQGTKVEIKR

SEQ ID NO: 267 - DNA, 18 bp, Artificial Sequence
  Synthetic
cagagcattggtagtagc

SEQ ID NO: 268 - protein, 6 aa, Artificial Sequence
  Synthetic
QSIGSS

SEQ ID NO: 269 - DNA, 9 bp, Artificial Sequence
  Synthetic
tatgcttcc

SEQ ID NO: 270 - protein, 3 aa, Artificial Sequence
  Synthetic
YAS

SEQ ID NO: 271 - DNA, 24 bp, Artificial Sequence
  Synthetic
cttcagagtagtagtttacggacg

SEQ ID NO: 272 - protein, 8 aa, Artificial Sequence
  Synthetic
LQSSSLRT

SEQ ID NO: 273 - DNA, 360 bp, Artificial Sequence
  Synthetic
gaggtgcagctggtggagtctgggggaggcttggtcaagcctggagggtccctgagactctcctgtgcagcctctggattcaccttcagtgactactacatgaactggatccgccaggctccagggaaggggctggagtggatttcatatcttagtagtagtggtagtgccacatactacgcagactctgtgaagggccgattcaccatctccagggacaacgccaagaactcactgtatctgcaaatgaacagcctgagagccgaggacacggccgtgtattattgtgcgagagatgggaagtacaacaccgtcgccggggactactggggccagggaaccacggtcaccgtctcctca

SEQ ID NO: 274 - protein, 120 aa, Artificial Sequence
  Synthetic
EVQLVESGGGLVKPGGSLRLSCAASGFTFSDYYMNWIRQAPGKGLEWISYLSSSGSATYYADSVKGRFTISRDNAKNSLYLQMNSLRAEDTAVYYCARDGKYNTVAGDYWGQGTTVTVSS

SEQ ID NO: 275 - DNA, 24 bp, Artificial Sequence
  Synthetic
ggattcaccttcagtgactactac

SEQ ID NO: 276 - protein, 8 aa, Artificial Sequence
  Synthetic
GFTFSDYY

SEQ ID NO: 277 - DNA, 24 bp, Artificial Sequence
  Synthetic
cttagtagtagtggtagtgccaca

SEQ ID NO: 278 - protein, 8 aa, Artificial Sequence
  Synthetic
LSSSGSAT

SEQ ID NO: 279 - DNA, 39 bp, Artificial Sequence
  Synthetic
gcgagagatgggaagtacaacaccgtcgccggggactac

SEQ ID NO: 280 - protein, 13 aa, Artificial Sequence
  Synthetic
ARDGKYNTVAGDY

SEQ ID NO: 281 - DNA, 324 bp, Artificial Sequence
  Synthetic
gacatccagttgacccagtctccatcctccctgtctgcatctgtaggagacagagtcaccatcacttgccgggcaagtcagggcattagaaatgatttaggctggtatcagcagaaaccagggaaagcccctaagcgcctgatctatgctgcatccagtttacaaagtggggtcccatcaaggttcagcggcagtggatctgggacagaattcactctcacaatcagcagcctgcagcctgaagattttgcaacttattactgtctacaacataatagttacccgtacacttttggccaggggaccaaggtagagatcaaacga

SEQ ID NO: 282 - protein, 108 aa, Artificial Sequence
  Synthetic
DIQLTQSPSSLSASVGDRVTITCRASQGIRNDLGWYQQKPGKAPKRLIYAASSLQSGVPSRFSGSGSGTEFTLTISSLQPEDFATYYCLQHNSYPYTFGQGTKVEIKR

SEQ ID NO: 283 - DNA, 18 bp, Artificial Sequence
  Synthetic
cagggcattagaaatgat

SEQ ID NO: 284 - protein, 6 aa, Artificial Sequence
  Synthetic
QGIRND

SEQ ID NO: 285 - DNA, 9 bp, Artificial Sequence
  Synthetic
gctgcatcc

SEQ ID NO: 286 - protein, 3 aa, Artificial Sequence
  Synthetic
AAS

SEQ ID NO: 287 - DNA, 27 bp, Artificial Sequence
  Synthetic
ctacaacataatagttacccgtacact

SEQ ID NO: 288 - protein, 9 aa, Artificial Sequence
  Synthetic
LQHNSYPYT

SEQ ID NO: 289 - DNA, 360 bp, Artificial Sequence
  Synthetic
gaggtgcagctggtggagtctgggggaggcttggtcaagcctggagggtccctgagactctcctgtgcagcctctggattcaccttcagtgactactacatgaactggatccgccaggctccagggaaggggctggagtggatttcatacattagtagtagtgatgataccacatactacgcagactctgtgaagggccgattcaccatatccagggacaacgccaagaactcactgtatctgcaaatgaacagcctgagagccgaggacacggccgtgtattattgtgcgagagatgggaagtacaacaccgtcgccggggaccactggggccagggaaccctggtcaccgtctcctca

SEQ ID NO: 290 - protein, 120 aa, Artificial Sequence
  Synthetic
EVQLVESGGGLVKPGGSLRLSCAASGFTFSDYYMNWIRQAPGKGLEWISYISSSDDTTYYADSVKGRFTISRDNAKNSLYLQMNSLRAEDTAVYYCARDGKYNTVAGDHWGQGTLVTVSS

SEQ ID NO: 291 - DNA, 24 bp, Artificial Sequence
  Synthetic
ggattcaccttcagtgactactac

SEQ ID NO: 292 - protein, 8 aa, Artificial Sequence
  Synthetic
GFTFSDYY

SEQ ID NO: 293 - DNA, 24 bp, Artificial Sequence
  Synthetic
attagtagtagtgatgataccaca

SEQ ID NO: 294 - protein, 8 aa, Artificial Sequence
  Synthetic
ISSSDDTT

SEQ ID NO: 295 - DNA, 39 bp, Artificial Sequence
  Synthetic
gcgagagatgggaagtacaacaccgtcgccggggaccac

SEQ ID NO: 296 - protein, 13 aa, Artificial Sequence
  Synthetic
ARDGKYNTVAGDH

SEQ ID NO: 297 - DNA, 321 bp, Artificial Sequence
  Synthetic
gaaattgtgatgacacagtctccagactttcagtctgtggctccaaaggagaaagtcaccatcacctgccgggccagtcagaacattggtagtagcttacactggtaccagcagaaaccagatcagtctccaaagctcctcatcaagtatgcttcccagtccttctcaggggtcccctcgaggttcagtggcagtggatctgggacagatttcaccctcaccatcaatagcctggaagctgaagatgctgcaacgtattactgtcttcagagttatactttaaggacgttcggccaagggaccaaggtggagatcaaacga

SEQ ID NO: 298 - protein, 107 aa, Artificial Sequence
  Synthetic
EIVMTQSPDFQSVAPKEKVTITCRASQNIGSSLHWYQQKPDQSPKLLIKYASQSFSGVPSRFSGSGSGTDFTLTINSLEAEDAATYYCLQSYTLRTFGQGTKVEIKR

SEQ ID NO: 299 - DNA, 18 bp, Artificial Sequence
  Synthetic
cagaacattggtagtagc

SEQ ID NO: 300 - protein, 6 aa, Artificial Sequence
  Synthetic
QNIGSS

SEQ ID NO: 301 - DNA, 9 bp, Artificial Sequence
  Synthetic
tatgcttcc

SEQ ID NO: 302 - protein, 3 aa, Artificial Sequence
  Synthetic
YAS

SEQ ID NO: 303 - DNA, 24 bp, Artificial Sequence
  Synthetic
cttcagagttatactttaaggacg

SEQ ID NO: 304 - protein, 8 aa, Artificial Sequence
  Synthetic
LQSYTLRT

SEQ ID NO: 305 - DNA, 345 bp, Artificial Sequence
  Synthetic
gaggtgcagctggtggagtctgggggaggcttggtacagcctggggggtccctgagactctcctgtgcagcctctggattcacctttagcagttatgccatgagctgggtccgccaggctccagggaaggggctggagtgggtctcagctattagtggtcgtggttataacgcagactacgcagactccgtgaagggccggttcaccatctccagggacaattccaagaacacgctgtatctgcaaatgaacagcctgagagccgaagacacggccgtatattactgtgcgaaattggaatactttgactactggggccagggaaccctggtcactgtctcctca

SEQ ID NO: 306 - protein, 115 aa, Artificial Sequence
  Synthetic
EVQLVESGGGLVQPGGSLRLSCAASGFTFSSYAMSWVRQAPGKGLEWVSAISGRGYNADYADSVKGRFTISRDNSKNTLYLQMNSLRAEDTAVYYCAKLEYFDYWGQGTLVTVSS

SEQ ID NO: 307 - DNA, 24 bp, Artificial Sequence
  Synthetic
ggattcacctttagcagttatgcc

SEQ ID NO: 308 - protein, 8 aa, Artificial Sequence
  Synthetic
GFTFSSYA

SEQ ID NO: 309 - DNA, 24 bp, Artificial Sequence
  Synthetic
attagtggtcgtggttataacgca

SEQ ID NO: 310 - protein, 8 aa, Artificial Sequence
  Synthetic
ISGRGYNA

SEQ ID NO: 311 - DNA, 24 bp, Artificial Sequence
  Synthetic
gcgaaattggaatactttgactac

SEQ ID NO: 312 - protein, 8 aa, Artificial Sequence
  Synthetic
AKLEYFDY

SEQ ID NO: 313 - DNA, 321 bp, Artificial Sequence
  Synthetic
gacatccagatgacccagtctccttccaccctgtctgcatctgtaggagacagagtcaccatcacttgccgggccagtcagagtattagtagctggttggcctggtatcagcagaaaccagggaaagcccctaagctcctgatctataaggcgtctagtttagaaagtggggtcccatcaaggttcagcggcagtggatctgggacagatttcactctcaccatcagcagcctgaggcctgaagattttgcaacttattactgccaacagtataatagttaccctctgactttcggcggagggaccaaggtggagatcaaa

SEQ ID NO: 314 - protein, 107 aa, Artificial Sequence
  Synthetic
DIQMTQSPSTLSASVGDRVTITCRASQSISSWLAWYQQKPGKAPKLLIYKASSLESGVPSRFSGSGSGTDFTLTISSLRPEDFATYYCQQYNSYPLTFGGGTKVEIK

SEQ ID NO: 315 - DNA, 18 bp, Artificial Sequence
  Synthetic
cagagtattagtagctgg

SEQ ID NO: 316 - protein, 6 aa, Artificial Sequence
  Synthetic
QSISSW

SEQ ID NO: 317 - DNA, 9 bp, Artificial Sequence
  Synthetic
aaggcgtct

SEQ ID NO: 318 - protein, 3 aa, Artificial Sequence
  Synthetic
KAS

SEQ ID NO: 319 - DNA, 27 bp, Artificial Sequence
  Synthetic
caacagtataatagttaccctctgact

SEQ ID NO: 320 - protein, 9 aa, Artificial Sequence
  Synthetic
QQYNSYPLT

SEQ ID NO: 321 - DNA, 345 bp, Artificial Sequence
  Synthetic
gaggtgcagctggtggagtctgggggaggcttggtacagcctggggggtccctgagactctcctgtgcagcctctggattcacctttagcacctatgccatgcactgggtccgccaggctccagggaaggggctggagtgggtctcaagtattagtggtcgtggtcgtaactcagaccacgcagactccgtgaagggccggttcaccatctccagagacaattccaagaacacgctctatctacaaatgaacagcctgagagccgaggacacggccgtatattactgtgcgaggaccgaatacttccaccactggggccagggcaccctggtcaccgtctcctca

SEQ ID NO: 322 - protein, 115 aa, Artificial Sequence
  Synthetic
EVQLVESGGGLVQPGGSLRLSCAASGFTFSTYAMHWVRQAPGKGLEWVSSISGRGRNSDHADSVKGRFTISRDNSKNTLYLQMNSLRAEDTAVYYCARTEYFHHWGQGTLVTVSS

SEQ ID NO: 323 - DNA, 24 bp, Artificial Sequence
  Synthetic
ggattcacctttagcacctatgcc

SEQ ID NO: 324 - protein, 8 aa, Artificial Sequence
  Synthetic
GFTFSTYA

SEQ ID NO: 325 - DNA, 24 bp, Artificial Sequence
  Synthetic
attagtggtcgtggtcgtaactca

SEQ ID NO: 326 - protein, 8 aa, Artificial Sequence
  Synthetic
ISGRGRNS

SEQ ID NO: 327 - DNA, 24 bp, Artificial Sequence
  Synthetic
gcgaggaccgaatacttccaccac

SEQ ID NO: 328 - protein, 8 aa, Artificial Sequence
  Synthetic
ARTEYFHH

SEQ ID NO: 329 - DNA, 321 bp, Artificial Sequence
  Synthetic
gacatccagatgacccagtctccatcctcactgtctgcatctgtaggagacagaatcaccatcacttgtcgggcgagtcaggacattaacaattatttagcctggtttcagcagaaaccaggaaaagcccctaagtccctgatctatggtgcatccagcttgcaaagtggggtcccatcaaagttcagcggcagtggatctgggacagatttcactctcaccatcagcagcctgcagcctgaagattttgcaacttattactgccaacaatatagttcttacccattcactttcggccctgggaccaaagtggatatcaaa

SEQ ID NO: 330 - protein, 107 aa, Artificial Sequence
  Synthetic
DIQMTQSPSSLSASVGDRITITCRASQDINNYLAWFQQKPGKAPKSLIYGASSLQSGVPSKFSGSGSGTDFTLTISSLQPEDFATYYCQQYSSYPFTFGPGTKVDIK

SEQ ID NO: 331 - DNA, 18 bp, Artificial Sequence
  Synthetic
caggacattaacaattat

SEQ ID NO: 332 - protein, 6 aa, Artificial Sequence
  Synthetic
QDINNY

SEQ ID NO: 333 - DNA, 9 bp, Artificial Sequence
  Synthetic
ggtgcatcc

SEQ ID NO: 334 - protein, 3 aa, Artificial Sequence
  Synthetic
GAS

SEQ ID NO: 335 - DNA, 27 bp, Artificial Sequence
  Synthetic
caacaatatagttcttacccattcact

SEQ ID NO: 336 - protein, 9 aa, Artificial Sequence
  Synthetic
QQYSSYPFT

SEQ ID NO: 337 - DNA, 348 bp, Artificial Sequence
  Synthetic
gaggtgcagctggtggagtctgggggaggcttggtccagcctggggggtccctgagactctcctgtgcagcctctggattcatctttagtacctattggatgaactgggtccgccaggctccagggaaggggctggagtgggtggccaacgtgaaccatgatggaagtgaggaatactatgtggactctgtgaagggccgattcaccatctccagagacaacgcccagaattcactgtatctgcaaatggaccgcctgagagccgaggacacggctatgtatttctgtgcgcgaagagccgggctttttgactcctggggccagggaaccctggtcactgtctcctca

SEQ ID NO: 338 - protein, 116 aa, Artificial Sequence
  Synthetic
EVQLVESGGGLVQPGGSLRLSCAASGFIFSTYWMNWVRQAPGKGLEWVANVNHDGSEEYYVDSVKGRFTISRDNAQNSLYLQMDRLRAEDTAMYFCARRAGLFDSWGQGTLVTVSS

SEQ ID NO: 339 - DNA, 24 bp, Artificial Sequence
  Synthetic
ggattcatctttagtacctattgg

SEQ ID NO: 340 - protein, 8 aa, Artificial Sequence
  Synthetic
GFIFSTYW

SEQ ID NO: 341 - DNA, 24 bp, Artificial Sequence
  Synthetic
gtgaaccatgatggaagtgaggaa

SEQ ID NO: 342 - protein, 8 aa, Artificial Sequence
  Synthetic
VNHDGSEE

SEQ ID NO: 343 - DNA, 27 bp, Artificial Sequence
  Synthetic
gcgcgaagagccgggctttttgactcc

SEQ ID NO: 344 - protein, 9 aa, Artificial Sequence
  Synthetic
ARRAGLFDS

SEQ ID NO: 345 - DNA, 321 bp, Artificial Sequence
  Synthetic
gacatccagatgacccagtctccatcttccgtgtctgcatctgtaggagacagagtcaccatcacttgtcgggcgagtcaggatattgacaactggttagcctggtatcagcagaaaccagggaaagcccctaaactcctgatctttacttcatccactttgcaaagtggggtcccatcaaggttcagcggcattggatctggaacagatttcactctcaccatcagcagcctacagcctgaagattttgcaacttactattgtcaacaggctaacagtttcccgtggacgttcggccaagggaccaaggtggagatcaaa

SEQ ID NO: 346 - protein, 107 aa, Artificial Sequence
  Synthetic
DIQMTQSPSSVSASVGDRVTITCRASQDIDNWLAWYQQKPGKAPKLLIFTSSTLQSGVPSRFSGIGSGTDFTLTISSLQPEDFATYYCQQANSFPWTFGQGTKVEIK

SEQ ID NO: 347 - DNA, 18 bp, Artificial Sequence
  Synthetic
caggatattgacaactgg

SEQ ID NO: 348 - protein, 6 aa, Artificial Sequence
  Synthetic
QDIDNW

SEQ ID NO: 349 - DNA, 9 bp, Artificial Sequence
  Synthetic
acttcatcc

SEQ ID NO: 350 - protein, 3 aa, Artificial Sequence
  Synthetic
TSS

SEQ ID NO: 351 - DNA, 27 bp, Artificial Sequence
  Synthetic
caacaggctaacagtttcccgtggacg

SEQ ID NO: 352 - protein, 9 aa, Artificial Sequence
  Synthetic
QQANSFPWT

SEQ ID NO: 353 - DNA, 375 bp, Artificial Sequence
  Synthetic
caggtgcagctggtggagtctgggggaggcgtggtcctgcctgggaggtccctgagactctcctgtgcagcgtctggattcacctttagtagttatctcatgtattgggtccgccaggctccaggcaaggggctggagtgggtggcagttatatggtatgatggaagtaataaattctatggagactccgtgaagggccgattcaccatctccagagacaattccaagaacacgttgtatctgcaaatgaacagcctgagagccgaggacacggctgtgtattactgtgcgagagataatgggaatagtggttacgaggacagctggaatgcttttgatatatggggccaagggacaatggtcaccgtctcttca

SEQ ID NO: 354 - protein, 125 aa, Artificial Sequence
  Synthetic
QVQLVESGGGVVLPGRSLRLSCAASGFTFSSYLMYWVRQAPGKGLEWVAVIWYDGSNKFYGDSVKGRFTISRDNSKNTLYLQMNSLRAEDTAVYYCARDNGNSGYEDSWNAFDIWGQGTMVTVSS

SEQ ID NO: 355 - DNA, 24 bp, Artificial Sequence
  Synthetic
ggattcacctttagtagttatctc

SEQ ID NO: 356 - protein, 8 aa, Artificial Sequence
  Synthetic
GFTFSSYL

SEQ ID NO: 357 - DNA, 24 bp, Artificial Sequence
  Synthetic
atatggtatgatggaagtaataaa

SEQ ID NO: 358 - protein, 8 aa, Artificial Sequence
  Synthetic
IWYDGSNK

SEQ ID NO: 359 - DNA, 54 bp, Artificial Sequence
  Synthetic
gcgagagataatgggaatagtggttacgaggacagctggaatgcttttgatata

SEQ ID NO: 360 - protein, 18 aa, Artificial Sequence
  Synthetic
ARDNGNSGYEDSWNAFDI

SEQ ID NO: 361 - DNA, 321 bp, Artificial Sequence
  Synthetic
gacatccagatgacccagtctccatcctcactgtctgcatctgtaggagacagagtcaccatcacttgtcgggcgagtcaggacatttacaattatttagcctggtttcagcagaaaccagggaaagcccctaagtccctgatctatgctgcatccagtttgcaaactggggtcccatcacagttcagcggcagtggatctgggacagatttcactctcaccatcagcagcctccagcctgaagattttgcaacttattactgccaacagtataataattacccattcactttcggccctgggaccaaagtggatatcaaa

SEQ ID NO: 362 - protein, 107 aa, Artificial Sequence
  Synthetic
DIQMTQSPSSLSASVGDRVTITCRASQDIYNYLAWFQQKPGKAPKSLIYAASSLQTGVPSQFSGSGSGTDFTLTISSLQPEDFATYYCQQYNNYPFTFGPGTKVDIK

SEQ ID NO: 363 - DNA, 18 bp, Artificial Sequence
  Synthetic
caggacatttacaattat

SEQ ID NO: 364 - protein, 6 aa, Artificial Sequence
  Synthetic
QDIYNY

SEQ ID NO: 365 - DNA, 9 bp, Artificial Sequence
  Synthetic
gctgcatcc

SEQ ID NO: 366 - protein, 3 aa, Artificial Sequence
  Synthetic
AAS

SEQ ID NO: 367 - DNA, 27 bp, Artificial Sequence
  Synthetic
caacagtataataattacccattcact

SEQ ID NO: 368 - protein, 9 aa, Artificial Sequence
  Synthetic
QQYNNYPFT

SEQ ID NO: 369 - DNA, 360 bp, Artificial Sequence
  Synthetic
gaggtgcagctggtggagtctgggggaggcttggcacagcctggggggtccctgagactctcctgtgcagcctctggattcacctttaacaactatgccatgacctgggtccgccaggctccagggaagggtctggactgggtctcagctattagtgatagtggtcgtagcacattctccgcagactccgtgaagggccggttcaccatctccagagacaactccaagaacacgctgtatctgcaaatggacagcctgagagccgaggacacggccttatattactgtgcgaaacataggaactggaactatcccgtctttgactactggggccagggaaccctggtcaccgtctcctca

SEQ ID NO: 370 - protein, 120 aa, Artificial Sequence
  Synthetic
EVQLVESGGGLAQPGGSLRLSCAASGFTFNNYAMTWVRQAPGKGLDWVSAISDSGRSTFSADSVKGRFTISRDNSKNTLYLQMDSLRAEDTALYYCAKHRNWNYPVFDYWGQGTLVTVSS

SEQ ID NO: 371 - DNA, 24 bp, Artificial Sequence
  Synthetic
ggattcacctttaacaactatgcc

SEQ ID NO: 372 - protein, 8 aa, Artificial Sequence
  Synthetic
GFTFNNYA

SEQ ID NO: 373 - DNA, 24 bp, Artificial Sequence
  Synthetic
attagtgatagtggtcgtagcaca

SEQ ID NO: 374 - protein, 8 aa, Artificial Sequence
  Synthetic
ISDSGRST

SEQ ID NO: 375 - DNA, 39 bp, Artificial Sequence
  Synthetic
gcgaaacataggaactggaactatcccgtctttgactac

SEQ ID NO: 376 - protein, 13 aa, Artificial Sequence
  Synthetic
AKHRNWNYPVFDY

SEQ ID NO: 377 - DNA, 321 bp, Artificial Sequence
  Synthetic
gacatccagttgacccagtctccatccttcctgtctgcatctgtgggagacagagtcaccatcacttgctgggccagtcagggcattagtagttatttagcctggtatcagcaaaaaccagggaaagccccaaagctcctgatctattctgcatccactttacaaagtggggtcccatcaaggttcagcggcagtggatctgggacagaattcactctcacaatcagcagcctgcagcctgaagattttgcaacttattactgtcaacaacttaatagttacccattcactttcggccctgggaccaaagtggatatcaaa

SEQ ID NO: 378 - protein, 107 aa, Artificial Sequence
  Synthetic
DIQLTQSPSFLSASVGDRVTITCWASQGISSYLAWYQQKPGKAPKLLIYSASTLQSGVPSRFSGSGSGTEFTLTISSLQPEDFATYYCQQLNSYPFTFGPGTKVDIK

SEQ ID NO: 379 - DNA, 18 bp, Artificial Sequence
  Synthetic
cagggcattagtagttat

SEQ ID NO: 380 - protein, 6 aa, Artificial Sequence
  Synthetic
QGISSY

SEQ ID NO: 381 - DNA, 9 bp, Artificial Sequence
  Synthetic
tctgcatcc

SEQ ID NO: 382 - protein, 3 aa, Artificial Sequence
  Synthetic
SAS

SEQ ID NO: 383 - DNA, 27 bp, Artificial Sequence
  Synthetic
caacaacttaatagttacccattcact

SEQ ID NO: 384 - protein, 9 aa, Artificial Sequence
  Synthetic
QQLNSYPFT

SEQ ID NO: 385 - protein, 190 aa, Artificial Sequence
  Synthetic
VKMAETCPIFYDVFFAVANGNELLLDLSLTKVNATEPERTAMKKIQDCYVENGLISRVLDGLVMTTISSSKDCMGEAVQNTVEDLKLNTLGREICPAVKRDVDLFLTGTPDEYVEQVAQYKALPVVLENARILKNCVDAKMTEEDKENALSVLDKIYTSPLCEQKLISEEDLGGEQKLISEEDLHHHHHH

SEQ ID NO: 386 - protein, 8 aa, Artificial Sequence
  Synthetic
  VARIANT (1)...(1): Xaa = Gly
  VARIANT (2)...(2): Xaa = Phe, Tyr or Gly
  VARIANT (3)...(3): Xaa = Thr or Ser
  VARIANT (4)...(4): Xaa = Phe or Ile
  VARIANT (5)...(5): Xaa = Ser, Arg, Thr, or Asn
  VARIANT (6)...(6): Xaa = Asn, Thr, Asp, or Ser
  VARIANT (7)...(7): Xaa = Tyr
  VARIANT (8)...(8): Xaa = Asn, Tyr, or Ala
XXXXXXXX

SEQ ID NO: 387 - protein, 8 aa, Artificial Sequence
  Synthetic
  VARIANT (1)...(1): Xaa = Ile
  VARIANT (2)...(2): Xaa = Tyr, Ser, or Asn
  VARIANT (3)...(3): Xaa = Tyr, Ser, Gly, Pro, or Asp
  VARIANT (4)...(4): Xaa = Asp, Arg, or Ser
  VARIANT (5)...(5): Xaa = Gly, Val, or Ser
  VARIANT (6)...(6): Xaa = Ser, Gly, Arg, or Tyr
  VARIANT (7)...(7): Xaa = Tyr, Arg, Thr, Ser, or Asn
  VARIANT (8)...(8): Xaa = Ile, Thr, Ala, Ser, or absent
XXXXXXXX

SEQ ID NO: 388 - protein, 16 aa, Artificial Sequence
  Synthetic
  VARIANT (1)...(1): Xaa = Ala
  VARIANT (2)...(2): Xaa = Lys or Arg
  VARIANT (3)...(3): Xaa = Arg, Gly, His, Ser, Asp, Leu, or Thr
  VARIANT (4)...(4): Xaa = Thr, Pro, Arg, Gly, or Glu
  VARIANT (5)...(5): Xaa = Leu, Val, Gly, Lys, Tyr, or Asn
  VARIANT (6)...(6): Xaa = Ser, Arg, Thr, Ala, Tyr, Phe, or Trp
  VARIANT (7)...(7): Xaa = Tyr, Gly, Arg, Ala, Asn, Asp, His, or Asn
  VARIANT (8)...(8): Xaa = Tyr, Thr, Ser, or His
  VARIANT (9)...(9): Xaa = Val, Ser, Ala, Phe, Pro, or absent
  VARIANT (10)...(10): Xaa = Met, Gly, Asp, Pro, Val, or absent
  VARIANT (11)...(11): Xaa = Asp, Tyr, Ser, Gly, Phe, or absent
  VARIANT (12)...(12): Xaa = Val, Asp, Phe, or absent
  VARIANT (13)...(13): Xaa = Phe, Asp, or absent
  VARIANT (14)...(14): Xaa = Phe, Tyr, or absent
  VARIANT (15)...(15): Xaa = Asp or absent
  VARIANT (16)...(16): Xaa = Tyr or absent
XXXXXXXXXXXXXXXX

SEQ ID NO: 389 - protein, 12 aa, Artificial Sequence
  Synthetic
  VARIANT (1)...(1): Xaa = Gln
  VARIANT (2)...(2): Xaa = Gly, Ser, or Asp
  VARIANT (3)...(3): Xaa = Ile or Val
  VARIANT (4)...(4): Xaa = Ser, Leu, Asn, or Gly
  VARIANT (5)...(5): Xaa = Asn, Tyr, Gly, or Ser
  VARIANT (6)...(6): Xaa = Tyr, Ser, Phe, or Trp
  VARIANT (7)...(7): Xaa = Ser or absent
  VARIANT (8)...(8): Xaa = Asn or absent
  VARIANT (9)...(9): Xaa = Asn or absent
  VARIANT (10)...(10): Xaa = Lys or absent
  VARIANT (11)...(11): Xaa = Gln or absent
  VARIANT (12)...(12): Xaa = Tyr or absent
XXXXXXXXXXXX

SEQ ID NO: 390 - protein, 3 aa, Artificial Sequence
  Synthetic
  VARIANT (1)...(1): Xaa = Ala, Trp, Asp, Tyr, Lys, Gly, or Ser
  VARIANT (2)...(2): Xaa = Ala or Thr
  VARIANT (3)...(3): Xaa = Ser
XXX

SEQ ID NO: 391 - protein, 9 aa, Artificial Sequence
  Synthetic
  VARIANT (1)...(1): Xaa = Gln, Leu, or His
  VARIANT (2)...(2): Xaa = Lys, Gln, or His
  VARIANT (3)...(3): Xaa = Tyr, Ser, or Leu
  VARIANT (4)...(4): Xaa = Tyr, Asn, Gly, Asp, or Ser
  VARIANT (5)...(5): Xaa = Ser, Asp, or Asn
  VARIANT (6)...(6): Xaa = Leu, Ala, Tyr, Thr, or Phe
  VARIANT (7)...(7): Xaa = Pro or Arg
  VARIANT (8)...(8): Xaa = Leu, Phe, Tyr, or Thr
  VARIANT (9)...(9): Xaa = Thr or absent
XXXXXXXXX

SEQ ID NO: 392 - protein, 70 aa, Artificial Sequence
  Synthetic
EICPAVKRDVDLFLTGTPDEYVEQVAQYKALPVVLENARILKNCVDAKMTEEDKENALSLLDKIYTSPLC

SEQ ID NO: 393 - protein, 92 aa, Artificial Sequence
  Synthetic
VKMAETCPIFYDVFFAVANGNELLLDLSLTKVNATEPERTAMKKIQDCYVENGLISRVLDGLVMTTISSSKDCMGEAVQNTVEDLKLNTLGR

SEQ ID NO: 394 - protein, 398 aa, Artificial Sequence
  Synthetic
VKMAETCPIFYDVFFAVANGNELLLDLSLTKVNATEPERTAMKKIQDCYVENGLISRVLDGLVMTTISSSKDCMGEAVQNTVEDLKLNTLGREICPAVKRDVDLFLTGTPDEYVEQVAQYKALPVVLENARILKNCVDAKMTEEDKENALSLLDKIYTSPLCLINEPRGPTIKPCPPCKCPAPNLLGGPSVFIFPPKIKDVLMISLSPIVTCVVVDVSEDDPDVQISWFVNNVEVHTAQTQTHREDYNSTLRVVSALPIQHQDWMSGKEFKCKVNNKDLPAPIERTISKPKGSVRAPQVYVLPPPEEEMTKKQVTLTCMVTDFMPEDIYVEWTNNGKTELNYKNTEPVLDSDGSYFMYSKLRVEKKNWVERNSYSCSVVHEGLHNHHTTKSFSRTPGK

SEQ ID NO: 395 - protein, 413 aa, Artificial Sequence
  Synthetic
EICPAVKRDVDLFLTGTPDEYVEQVAQYKALPVVLENARILKNCVDAKMTEEDKENALSLLDKIYTSPLCGGGGSGGGGSGGGGSVKMAETCPIFYDVFFAVANGNELLLDLSLTKVNATEPERTAMKKIQDCYVENGLISRVLDGLVMTTISSSKDCMGEAVQNTVEDLKLNTLGRLINEPRGPTIKPCPPCKCPAPNLLGGPSVFIFPPKIKDVLMISLSPIVTCVVVDVSEDDPDVQISWFVNNVEVHTAQTQTHREDYNSTLRVVSALPIQHQDWMSGKEFKCKVNNKDLPAPIERTISKPKGSVRAPQVYVLPPPEEEMTKKQVTLTCMVTDFMPEDIYVEWTNNGKTELNYKNTEPVLDSDGSYFMYSKLRVEKKNWVERNSYSCSVVHEGLHNHHTTKSFSRTPGK

SEQ ID NO: 396 - protein, 199 aa, Artificial Sequence
  Synthetic
VKMAETCPIFYDVFFAVANGNELLLDLSLTKVNATEPERTAMKKIQDCYVENGLISRVLDGLVMTTISSSKDCMGEAVQNTVEDLKLNTLGREICPAVKRGVDLFLTGTPDEYVEQVAQYKALPVVLENARILKNCVDAKMTEEDKENALSLLDKIYTSPLCGPGGEQKLISEEDLGGEQKLISEEDLSGHHHHHHSSG

SEQ ID NO: 397 - protein, 214 aa, Artificial Sequence
  Synthetic
EICPAVKRDVDLFLTGTPDEYVEQVAQYKALPVVLENARILKNCVDAKMTEEDKENALSLLDKIYTSPLCGGGGSGGGGSGGGGSVKMAETCPIFYDVFFAVANGNELLLDLSLTKVNATEPERTAMKKIQDCYVENGLISRVLDGLVMTTISSSKDCMGEAVQNTVEDLKLNTLGRGPGGEQKLISEEDLGGEQKLISEEDLSGHHHHHHSSG

SEQ ID NO: 398 - protein, 11 aa, Artificial Sequence
  Synthetic
VKMAETCPIFY

SEQ ID NO: 399 - protein, 7 aa, Artificial Sequence
  Synthetic
ISRVLDG

SEQ ID NO: 400 - protein, 8 aa, Artificial Sequence
  Synthetic
ISRVLDGL

SEQ ID NO: 401 - protein, 10 aa, Artificial Sequence
  Synthetic
ISRVLDGLVM

SEQ ID NO: 402 - protein, 19 aa, Artificial Sequence
  Synthetic
LKLNTLGREICPAVKRGVD

SEQ ID NO: 403 - protein, 20 aa, Artificial Sequence
  Synthetic
LKLNTLGREICPAVKRGVDL

SEQ ID NO: 404 - protein, 15 aa, Artificial Sequence
  Synthetic
YVEQVAQYKALPVVL

SEQ ID NO: 405 - protein, 11 aa, Artificial Sequence
  Synthetic
VAQYKALPVVL

SEQ ID NO: 406 - protein, 14 aa, Artificial Sequence
  Synthetic
ENARILKNCVDAKM

SEQ ID NO: 407 - protein, 18 aa, Artificial Sequence
  Synthetic
LDKIYTSPLCGPGGEQKL

SEQ ID NO: 408 - protein, 14 aa, Artificial Sequence
  Synthetic
ISEEDLSGHHHHHH

SEQ ID NO: 409 - protein, 17 aa, Artificial Sequence
  Synthetic
ISEEDLSGHHHHHHSSG

SEQ ID NO: 410 - protein, 14 aa, Artificial Sequence
  Synthetic
EDLSGHHHHHHSSG

SEQ ID NO: 411 - protein, 11 aa, Artificial Sequence
  Synthetic
VKMAETCPIFY

SEQ ID NO: 412 - protein, 10 aa, Artificial Sequence
  Synthetic
FAVANGNELL

SEQ ID NO: 413 - protein, 7 aa, Artificial Sequence
  Synthetic
ISRVLDG

SEQ ID NO: 414 - protein, 8 aa, Artificial Sequence
  Synthetic
ISRVLDGL

SEQ ID NO: 415 - protein, 10 aa, Artificial Sequence
  Synthetic
ISRVLDGLVM

SEQ ID NO: 416 - protein, 19 aa, Artificial Sequence
  Synthetic
LKLNTLGREICPAVKRGVD

SEQ ID NO: 417 - protein, 20 aa, Artificial Sequence
  Synthetic
LKLNTLGREICPAVKRGVDL

SEQ ID NO: 418 - protein, 15 aa, Artificial Sequence
  Synthetic
YVEQVAQYKALPVVL

SEQ ID NO: 419 - protein, 11 aa, Artificial Sequence
  Synthetic
VAQYKALPVVL

SEQ ID NO: 420 - protein, 8 aa, Artificial Sequence
  Synthetic
YKALPVVL

SEQ ID NO: 421 - protein, 14 aa, Artificial Sequence
  Synthetic
ENARILKNCVDAKM

SEQ ID NO: 422 - protein, 18 aa, Artificial Sequence
  Synthetic
LDKIYTSPLCGPGGEQKL

SEQ ID NO: 423 - protein, 14 aa, Artificial Sequence
  Synthetic
ISEEDLSGHHHHHH

SEQ ID NO: 424 - protein, 17 aa, Artificial Sequence
  Synthetic
ISEEDLSGHHHHHHSSG

SEQ ID NO: 425 - protein, 14 aa, Artificial Sequence
  Synthetic
EDLSGHHHHHHSSG

SEQ ID NO: 426 - protein, 4 aa, Artificial Sequence
  Synthetic
YVEQ

SEQ ID NO: 427 - DNA, 363 bp, Artificial Sequence
  Synthetic
gaggtgcagctggtggagtcgggcccaggactggtgaacccttcggagaccctgtccctcacctgctctgtctctggtggctccatcagcagtgttaattactactggggctggatccgccagtccccagggaagggactggagtggattgggagtatctattatactgggagtaccgactacaacccgtccctcaagaatcgagtcaccatatccgtagacacgtccaagaaccagttctccctgaagcagacttctgtgaccgccgcagacacggctgtctattactgtgcgagacatgtggcactggctggggggcttttgatagtctggggccaggggacaatggtcaccgtctcttca

SEQ ID NO: 428 - protein, 121 aa, Artificial Sequence
  Synthetic
EVQLVESGPGLVNPSETLSLTCSVSGGSISSVNYYWGWIRQSPGKGLEWIGSIYYTGSTDYNPSLKNRVTISVDTSKNQFSLKQTSVTAADTAVYYCARHVALAGGLLIVWGQGTMVTVSS

SEQ ID NO: 429 - DNA, 30 bp, Artificial Sequence; identical to SEQ ID NO: 179
  Synthetic

SEQ ID NO: 430 - protein, 10 aa, Artificial Sequence
  Synthetic
GGSISSVNYY

SEQ ID NO: 431 - DNA, 21 bp, Artificial Sequence
  Synthetic
atctattatactgggagtacc

SEQ ID NO: 432 - protein, 7 aa, Artificial Sequence
  Synthetic
IYYTGST

SEQ ID NO: 433 - DNA, 39 bp, Artificial Sequence
  Synthetic
gcgagacatgtggcactggctggggggcttttgatagtc

SEQ ID NO: 434 - protein, 13 aa, Artificial Sequence
  Synthetic
ARHVALAGGLLIV

SEQ ID NO: 435 - DNA, 342 bp, Artificial Sequence
  Synthetic
gacatccagatgacccagtctccagactccctggctgtgtctctgggcgcgagggccaccatcaactgcaagtccagccaaagtgttttattcagctccaacaataagaacttcttagcctggtaccagcagaaaccaggacagcctcctaccctgctcatttcctgggcatctacccgggaatccggggtccctgaccgattcagtgggagcgggtctgggacagatttcactctcaccatcagcagcctgcaggctgaagatgtggcagtttatttctgtcaacaatattataatagtcctccacttttcggccaggggaccaaggtggagatcaaacga

SEQ ID NO: 436 - protein, 114 aa, Artificial Sequence
  Synthetic
DIQMTQSPDSLAVSLGARATINCKSSQSVLFSSNNKNFLAWYQQKPGQPPTLLISWASTRESGVPDRFSGSGSGTDFTLTISSLQAEDVAVYFCQQYYNSPPLFGQGTKVEIKR

SEQ ID NO: 437 - DNA, 36 bp, Artificial Sequence
  Synthetic
caaagtgttttattcagctccaacaataagaacttc

SEQ ID NO: 438 - protein, 12 aa, Artificial Sequence
  Synthetic
QSVLFSSNNKNF

SEQ ID NO: 439 - DNA, 9 bp, Artificial Sequence
  Synthetic
tgggcatct

SEQ ID NO: 440 - protein, 3 aa, Artificial Sequence
  Synthetic
WAS

SEQ ID NO: 441 - DNA, 27 bp, Artificial Sequence
  Synthetic
caacaatattataatagtcctccactt

SEQ ID NO: 442 - protein, 9 aa, Artificial Sequence
  Synthetic
QQYYNSPPL

SEQ ID NO: 443 - DNA, 360 bp, Artificial Sequence
  Synthetic
gaggtgcagctggtggagtctgggggaggcttggtacagcctggggggtccctgagactctcctgtgcagtctctggattcacctttagcaactatgccatgaactgggtccgccaggctccagggaaggggctggagtgggtctcagttattagcgacagtggtcgtagcacctactacgcagactccgtgaagggccggttcaccatctccagagacaattccaagaacacgctatatctgcaaatgaacagcctgagagccgaggacacggccgtatatttctgtgcgaaaaggtataactggaacttacactactttgactactggggccagggaaccacggtcaccgtctcctca

SEQ ID NO: 444 - protein, 120 aa, Artificial Sequence
  Synthetic
EVQLVESGGGLVQPGGSLRLSCAVSGFTFSNYAMNWVRQAPGKGLEWVSVISDSGRSTYYADSVKGRFTISRDNSKNTLYLQMNSLRAEDTAVYFCAKRYNWNLHYFDYWGQGTTVTVSS

SEQ ID NO: 445 - DNA, 24 bp, Artificial Sequence
  Synthetic
ggattcacctttagcaactatgcc

SEQ ID NO: 446 - protein, 8 aa, Artificial Sequence
  Synthetic
GFTFSNYA

SEQ ID NO: 447 - DNA, 24 bp, Artificial Sequence
  Synthetic
attagcgacagtggtcgtagcacc

SEQ ID NO: 448 - protein, 8 aa, Artificial Sequence
  Synthetic
ISDSGRST

SEQ ID NO: 449 - DNA, 39 bp, Artificial Sequence
  Synthetic
gcgaaaaggtataactggaacttacactactttgactac

SEQ ID NO: 450 - protein, 13 aa, Artificial Sequence
  Synthetic
AKRYNWNLHYFDY

SEQ ID NO: 451 - DNA, 321 bp, Artificial Sequence
  Synthetic
gaaattgtgttgacgcagtctccagactttcagtctgtgactccaaaggagaaagtcaccatcacctgccgggccagtcagagcattggtggtagcttacactggtaccagcagaaaccagatcagtctccaaagctcctcatcaagtatgcttcccagtccttctcaggggtcccctcgaggttcagtggcagtggatctgggacagatttcaccctcaccatcaatagcctggaagctgaagatgctgcaacgtattactgtcttcagagtagtagtttacggacgttcggccaagggaccaaggtggagatcaaacga

SEQ ID NO: 452 - protein, 107 aa, Artificial Sequence
  Synthetic
EIVLTQSPDFQSVTPKEKVTITCRASQSIGGSLHWYQQKPDQSPKLLIKYASQSFSGVPSRFSGSGSGTDFTLTINSLEAEDAATYYCLQSSSLRTFGQGTKVEIKR

SEQ ID NO: 453 - DNA, 18 bp, Artificial Sequence
  Synthetic
cagagcattggtggtagc

SEQ ID NO: 454 - protein, 6 aa, Artificial Sequence
  Synthetic
QSIGGS

SEQ ID NO: 455 - DNA, 9 bp, Artificial Sequence
  Synthetic
tatgcttcc

SEQ ID NO: 456 - protein, 3 aa, Artificial Sequence
  Synthetic
YAS

SEQ ID NO: 457 - DNA, 24 bp, Artificial Sequence
  Synthetic
cttcagagtagtagtttacggacg

SEQ ID NO: 458 - protein, 8 aa, Artificial Sequence
  Synthetic
LQSSSLRT

SEQ ID NO: 459 - DNA, 345 bp, Artificial Sequence
  Synthetic
gaggtgcagctggtggagtctgggggaggcttggtacagcctggggggtccctgagactctcctgtgcagcctctggattcacctttagcagttatgccatgagctgggtccgccaggctccagggaaggggctggagtgggtctcagctattagtggtcgtggttataacgcagactacgcagactccgtgaagggccggttcaccatctccagagacaattccaagaacacgctgtatctgcaaatgaacagcctgagagccgaagacacggccgtatattactgtgcgaaattggaatactttgactactggggccagggaaccacggtcaccgtctcctca

SEQ ID NO: 460 - protein, 115 aa, Artificial Sequence
  Synthetic
EVQLVESGGGLVQPGGSLRLSCAASGFTFSSYAMSWVRQAPGKGLEWVSAISGRGYNADYADSVKGRFTISRDNSKNTLYLQMNSLRAEDTAVYYCAKLEYFDYWGQGTTVTVSS

SEQ ID NO: 461 - DNA, 24 bp, Artificial Sequence
  Synthetic
ggattcacctttagcagttatgcc

SEQ ID NO: 462 - protein, 8 aa, Artificial Sequence
  Synthetic
GFTFSSYA

SEQ ID NO: 463 - DNA, 24 bp, Artificial Sequence
  Synthetic
attagtggtcgtggttataacgca

SEQ ID NO: 464 - protein, 8 aa, Artificial Sequence
  Synthetic
ISGRGYNA

SEQ ID NO: 465 - DNA, 24 bp, Artificial Sequence
  Synthetic
gcgaaattggaatactttgactac

SEQ ID NO: 466 - protein, 8 aa, Artificial Sequence
  Synthetic
AKLEYFDY

SEQ ID NO: 467 - DNA, 324 bp, Artificial Sequence
  Synthetic
gacatccagttgacccagtctccttccaccctgtctgcatctgtaggagacagagtcaccatcacttgccgggccagtcagagtattagtagctggttggcctggtatcagcagaaaccagggaaagcccctaagctcctgatctataaggcgtctagtttagaaagtggggtcccatcaaggttcagcggcagtggatctgggacagatttcactctcaccatcagcagcctgaggcctgaagattttgcaacttattactgccaacagtataatagttaccctctgactttcggcggagggaccaaggtggaaatcaaacga

SEQ ID NO: 468 - protein, 108 aa, Artificial Sequence
  Synthetic
DIQLTQSPSTLSASVGDRVTITCRASQSISSWLAWYQQKPGKAPKLLIYKASSLESGVPSRFSGSGSGTDFTLTISSLRPEDFATYYCQQYNSYPLTFGGGTKVEIKR

SEQ ID NO: 469 - DNA, 18 bp, Artificial Sequence
  Synthetic
cagagtattagtagctgg

SEQ ID NO: 470 - protein, 6 aa, Artificial Sequence
  Synthetic
QSISSW

SEQ ID NO: 471 - DNA, 9 bp, Artificial Sequence
  Synthetic
aaggcgtct

SEQ ID NO: 472 - protein, 3 aa, Artificial Sequence
  Synthetic
KAS

SEQ ID NO: 473 - DNA, 27 bp, Artificial Sequence
  Synthetic
caacagtataatagttaccctctgact

SEQ ID NO: 474 - protein, 9 aa, Artificial Sequence
  Synthetic
QQYNSYPLT

SEQ ID NO: 475 - DNA, 345 bp, Artificial Sequence
  Synthetic
gaggtgcagctggtggagtctgggggaggcttggtacagcctggggggtccctgagactctcctgtgcagcctctggattcacctttagcacctatgccatgcactgggtccgccaggctccagggaaggggctggagtgggtctcaagtattagtggtcgtggtcgtaactcagaccacgcagactccgtgaagggccggttcaccatctccagagacaattccaagaacacgctctatctacaaatgaacagcctgagagccgaggacacggccgtatattactgtgcgaggaccgaatacttccaccactggggccagggcaccacggtcaccgtctcctca

SEQ ID NO: 476 - protein, 115 aa, Artificial Sequence
  Synthetic
EVQLVESGGGLVQPGGSLRLSCAASGFTFSTYAMHWVRQAPGKGLEWVSSISGRGRNSDHADSVKGRFTISRDNSKNTLYLQMNSLRAEDTAVYYCARTEYFHHWGQGTTVTVSS

SEQ ID NO: 477 - DNA, 24 bp, Artificial Sequence
  Synthetic
ggattcacctttagcacctatgcc

SEQ ID NO: 478 - protein, 8 aa, Artificial Sequence
  Synthetic
GFTFSTYA

SEQ ID NO: 479 - DNA, 24 bp, Artificial Sequence
  Synthetic
attagtggtcgtggtcgtaactca

SEQ ID NO: 480 - protein, 8 aa, Artificial Sequence
  Synthetic
ISGRGRNS

SEQ ID NO: 481 - DNA, 24 bp, Artificial Sequence
  Synthetic
gcgaggaccgaatacttccaccac

SEQ ID NO: 482 - protein, 8 aa, Artificial Sequence
  Synthetic
ARTEYFHH

SEQ ID NO: 483 - DNA, 324 bp, Artificial Sequence
  Synthetic
gacatcgtgatgacccagtctccatcctcactgtctgcatctgtaggagacagaatcaccatcacttgtcgggcgagtcaggacattaacaattatttagcctggtttcagcagaaaccaggaaaagcccctaagtccctgatctatggtgcatccagcttgcaaagtggggtcccatcaaagttcagcggcagtggatctgggacagatttcactctcaccatcagcagcctgcagcctgaagattttgcaacttattactgccaacaatatacgttcttaccattcactttcggccctgggaccaaggtgaaaatcaaacga

SEQ ID NO: 484 - protein, 108 aa, Artificial Sequence
  Synthetic
DIVMTQSPSSLSASVGDRITITCRASQDINNYLAWFQQKPGKAPKSLIYGASSLQSGVPSKFSGSGSGTDFTLTISSLQPEDFATYYCQQYTFLPFTFGPGTKVKIKR

SEQ ID NO: 485 - DNA, 18 bp, Artificial Sequence
  Synthetic
caggacattaacaattat

SEQ ID NO: 486 - protein, 6 aa, Artificial Sequence
  Synthetic
QDINNY

SEQ ID NO: 487 - DNA, 9 bp, Artificial Sequence
  Synthetic
ggtgcatcc

SEQ ID NO: 488 - protein, 3 aa, Artificial Sequence
  Synthetic
GAS

SEQ ID NO: 489 - DNA, 27 bp, Artificial Sequence
  Synthetic
caacaatatacgttcttaccattcact

SEQ ID NO: 490 - protein, 9 aa, Artificial Sequence
  Synthetic
QQYTFLPFT